European Patent Application EP 4 516 902 A1, published March 5, 2025. Title: ENO1 GENE PROMOTOR. Applicant: Daiichi Sankyo Company, Limited. Application JP. The sequence listing filed with the application follows.

SEQUENCE LISTING (18 sequences)

SEQ ID NO: 1 - DNA, 3003 bp, Cricetulus griseus
  source 1..3003: mol_type = genomic DNA
ggcacgcagcgcgcaggcgcggtgtcccacacccccctccccgcgccgcgttccacgcgagtgaggctcccacgctgcggcttaacgtttccacgccgctggggtctcccacacctcggggcggggccgggccgcgaaggtcaccaccaaggtcgagagccggacgtgctcgccgcctccaagccgagtgcgtgtgggactcggagtacgtgcggcgggccggagcccgcatgtcggctgcgtagcgacgccccgccctcacccagactccgcagaccctcagctcagcccccggctagcaacgggaggctcgcccagtaggccgaaaatgccacaggcccagccaaccaagtctacccccgcccccgggccatcgtcctcagactgtccgagccaggaggacacctcagtcacgctcttcttctggagtgacagcgccgggggccaatgcccggacggagaggacagagggcgggcccgaaacgccaagaatgggcgggccctcccgagctgctcacaaagtcggagtgggaggcgcttagaccagctcgggaaccggctcgtgcgcacgtccctgctaaacgctctccagggtgtgtataggaacctctgttcttttcctgctcgcccaccggagtgccaggtagggatcgggggcccctggggaacggttcgctcacgagctccgcgtggggggccccggtgggtgtgtgtgcgcccctccagcctgggcgcgtgcccggggactcgggaagcgttcggggcagcctcgtggagggacgtgggctcttggagggggctggggaggtgcagatccacctgttagcatccagacacaggcttgcagggcaactgggctcccaagcctacaaccgcaagtgcagaacagggtggatcgccgcccgggggggttagctaactggaggaaggctttttttttttttttttttttttgagggggagaatgatttgacctaatgctcaggaaaaaccttcacaaaatggaagggcctgaaagaaggatgcccaagaggcggtccctcgtcatcgtccgcctcccccccccccccccccgggctgctcgcagatcctgctagggctgtggctcatggaccgcaatctagcgtcactgggcgggagtggtccagcccatctctgccacggaatatactccggtgcttattctaggggaaattgcagcagaacccctggatagctggggagggcttaggcgacctcgccccagttaggcaagagttgcgggcttcctgagtggctgctagcaggccgagaaccgacttaggatgtgtttcaggaaatttcctgtcgcccctggcgtaagcagcgtggtccttttgctttcgtgggaggccagagccggcctgggcggatactttgacctctaggtccactattctgccccggctccggccttcagtccacttaaaagacctagagggtgagatttttatcctgggcaaagacagtgcagcccaacttagggatccgagtcagatgcatgctggaaggggagaaccaactcctacacgttagcctgacttcctagtgcgcgctggcacgtgggcgctcccccggcccaaatagatgaaaagaaaactaaagggccattgtgccagacaaggtgatgcgcacatataaacccggcacagggggcgctgcgacaggaggatcacttgagttcgggtcaacccggtatacataggacgtgggggtgggagaagacaaagaagtaaatggtatttaggcccagactgttatacaaaagtgtatttgaagtctacatagtaaatcattggtgttttaagatggaggttttttgtaacatagaggggtaaaaagtagatacttttcttgattagggtgtaaagatcctttgtctcacacaagacaaagcaacagaagaagctactcagttgaaacaaaaagatgcctttgcagcttcggcccttgccgtacgagacgtggagaacccagttagataaagatagtttatgaacaataatttagtttctcacctcatccaatttattgctaagagtttttttggtaaaattctgtcttggaaggcctactggggaaaaagtaagggattttaaacctctttagtgttgtggccatttcttaaaaatgagctaaaatgccctttttgaaagaaatatgattcagaagccatcagaggatcttaaatatggcggtgaggatggaacccattgctgcccacgtgctaggcaagctagcagacacgtgccagcagaccagaaagtgtagcgctgatgatcacagacgaaggacttacgtggtgctgccatccaagcccaatttctcaaactaactgaacatgcttctgttgccatgggtataatataacataggctgggtggttttttgttttgttttgttttttgcctaattttacatggtttatcctgtgaccttcacagcatcatcctacttcctttgcattaggccttgagtgtaaccagcccattgctctacccagtcggagaactgatggttttagtttggggttttttatgggttttgccctagtggttacaaaacaggttttttcttctccttagcactacatgctaagaacacatttgttaccatcccgcccgctctgggatttgtatggaagccagggtgttgagcatgccacttgagcactaagccatgaccttagcctcccacctgcttttgtacaaaagcgtagtttttactgatttgagatgcaccacagtgcacttgggtttgggaacacatttgtaggagtggttttgttgcaccaagtgatcatcaggcctgatttggatggcgcctggcttgaattttatgggatagttctagaggccctgcagcagcccacaccatcctgcccactgcttcaccgataagtccagaattcctcagaagtgatctcttgaaagtgttaaggtttgtggaaaatgtgaattgttttttttttttcccctacagaca

SEQ ID NO: 2 - DNA, 3000 bp, Mus musculus
  source 1..3000: mol_type = genomic DNA
gagctggacagtaggattcggtaccctccacacagtaacaaatgattaggtaatattaagggaaaggtcactttcccttggctacctcggcctgagactcactacagcaaggacaaaaggacggggtcaccttggcagatggcaccagagagccaggaccagcggcgagggcgctcagtgcgcaggcgcagtatccatgcatttccccctcatcccccccacccccacccaattccacgcgggagtgaggccctctggccgcgcatcaacgtttccacaccgccgggggctccagaacctcccggtggggggttggccggctggagggccgagccgcgaaggtcatcagcaaggtcgtgggccggacgtgtggcgccgcagccacgccgagtgcgtgtgagactcggagtacgtgcggcgggctcaagccctcatgcccgccgcgcagcccagccccgccccgccccgcatccgggctccgtagaccctcggccgggccccaggttcccagccggaggctcgccaggcattccagctatgccccaagcaggctaggcccagaaaggcaggacaacccccgcccccgtgccctcgcccctagtctgggcaggccgagcggccgcctcggtcacgctcttctattggagtgatggcacgctgagccaatggggaggcggcgcggagggagggcgggcccgaaaggggagaactgggcggggcttaacgagcaggaaaggaagacagagtgggaggcgcttagtgctgctccggtacagggtcgcgctcgcgtctgtccttaaggctctcctcggtgtccacggcaccctctttccttgctttgcagcgatcctactgccaggtatggtccttgtctccaccggggtcagctctcctactagcttcgcttggggacccggtgggcacgtgcacccactagcctgggcgggagccgctatccggggagcactcgggtcagcctcgtggaaggacgcaggctcttggagggtggaggtgtgagccccaccagtgatcaccgagtttcagggttgcaatgtaaccgggttcccaagcagacaacagcaaatgcagaccacggatgatcgcggccgtggagaatagaaaagtactttctgtgtagttaagtggaaggtttcagagggagggagagcaacttaaacccccgatgctcattaaatcctttctcagaatggaagggccagaaataaggatgcccaagaggcagagcgccacaccctagtagatcctgctggggctgtagctcctggaccgcaatcgagcgtcactgggcgggagtggtccagcccatctctgctgtggaatattcctgacctgtgagtgtcggttaggtactaagagtagaggaaattgcagcagtcccgttggataattgggaagccctcaggagacctcgacgcaattaggcaagagctacaggtttcctgggtggctactagccggccgtgaactgacttaagatgcatttaagaaaacttcctgttcgttctggcctaggcagtgtggttccttggctgactcgctttcgggatagaccacagctagtctgctgattagcctgaccgataggtccacttttctgcccttggtctggcgttcaatccagataaagacagagtgggtgagattttcttcctttggttaaatacgtttgctgcctagcctaaagatccaagctagataaaaagggtggagggagggatcaactcctacaagttgtaaggtctttgcagagcaaagtgtggcacgtgggtgctcctccgcccccataaaggaaccagccatggagatgcacacatgaaagtgtagcgctagggatgctgaggctggaggatcactgagttctggtcagtctggcattcatagaatcgggcgagtaagagagaagacaaaagagtatggttgaggaatagtaaggttttgtaacatggtaggtaaaaagtagatactttattcttggtgagtgtacaaagatcctttgtcttagagaagacaaaaccacagaagtaacttctgtggaaaaaaaagctgcctttgcttcagtgcttgccacaaaagatgtgaggaacctagttagataataatagcctctgaatgctgtattgtcttcatgtctcatccagtttagctacagaatctatttggtttctttcttggaaagcctgctggggaagaagtaagaaagggacttgcagtttgttgccaaatatcctcttcctctcaggatgtttttctaattaaacatctactttgaataccttttaaaagcgagacaaggtgcccttttgaaatgtactaaccagaagtcctagctcttgcctaaatatggcggagattgaacccaggacctcccacgtgctagccagcatggccaccaggccaagaatggcaggatcattgaccacaggccaaggagtttggggttctggcctcctgcctcacactttcttactggttatcaaatctgtgtcagctgaatattctgctcttgtcatgggtgcaatttgatgaattagggtttctctttttcccacaattaaactgctttgaaatgtcacatttccctctggtctccaggtcagtttaacctctgaccttccttcactgttgcttcccacttccttctctgtggagccagaacactgttctatgcagtcagaggatttaatttgcccacagtacaggtagcttctgagggctttctgtaggagtggtttatttcattgtgccatgttgacctcaagcttggcgggaagtccaagccaccgacctgctgtgtaaggagtagtcctcgctccccaaaccctcactgatgagtgactttcctgtatgttacctaacgcatagcccatttggtacctgtcaagtccaggacccctcagaggtgatggccttggaatgaattaacctctgtgtcactgtttattggtgatatgaatgtttttcctcctacagaaattcgcc

SEQ ID NO: 3 - DNA, 2807 bp, Cricetulus griseus
  source 1..2807: mol_type = genomic DNA
gtgggactcggagtacgtgcggcgggccggagcccgcatgtcggctgcgtagcgacgccccgccctcacccagactccgcagaccctcagctcagcccccggctagcaacgggaggctcgcccagtaggccgaaaatgccacaggcccagccaaccaagtctacccccgcccccgggccatcgtcctcagactgtccgagccaggaggacacctcagtcacgctcttcttctggagtgacagcgccgggggccaatgcccggacggagaggacagagggcgggcccgaaacgccaagaatgggcgggccctcccgagctgctcacaaagtcggagtgggaggcgcttagaccagctcgggaaccggctcgtgcgcacgtccctgctaaacgctctccagggtgtgtataggaacctctgttcttttcctgctcgcccaccggagtgccaggtagggatcgggggcccctggggaacggttcgctcacgagctccgcgtggggggccccggtgggtgtgtgtgcgcccctccagcctgggcgcgtgcccggggactcgggaagcgttcggggcagcctcgtggagggacgtgggctcttggagggggctggggaggtgcagatccacctgttagcatccagacacaggcttgcagggcaactgggctcccaagcctacaaccgcaagtgcagaacagggtggatcgccgcccgggggggttagctaactggaggaaggctttttttttttttttttttttgagggggagaatgatttgacctaatgctcaggaaaaaccttcacaaaatggaagggcctgaaagaaggatgcccaagaggcggtccctcgtcatcgtccgcctccccccccccccccccgggctgctcgcagatcctgctagggctgtggctcatggaccgcaatctagcgtcactgggcgggagtggtccagcccatctctgccacggaatatactccggtgcttattctaggggaaattgcagcagaacccctggatagctggggagggcttaggcgacctcgccccagttaggcaagagttgcgggcttcctgagtggctgctagcaggccgagaaccgacttaggatgtgtttcaggaaatttcctgtcgcccctggcgtaagcagcgtggtccttttgctttcgtgggaggccagagccggcctgggcggatactttgacctctaggtccactattctgccccggctccggccttcagtccacttaaaagacctagagggtgagatttttatcctgggcaaagacagtgcagcccaacttagggatccgagtcagatgcatgctggaaggggagaaccaactcctacacgttagcctgacttcctagtgcgcgctggcacgtgggcgctcccccggcccaaatagatgaaaagaaaactaaagggccattgtgccagacaaggtgatgcgcacatataaacccggcacagggggcgctgcgacaggaggatcacttgagttcgggtcaacccggtatacataggacgtgggggtgggagaagacaaagaagtaaatggtatttaggcccagactgttatacaaaagtgtatttgaagtctacatagtaaatcattggtgttttaagatggaggttttttgtaacatagaggggtaaaaagtagatacttttcttgattagggtgtaaagatcctttgtctcacacaagacaaagcaacagaagaagctactcagttgaaacaaaaagatgcctttgcagcttcggcccttgccgtacgagacgtggagaacccagttagataaagatagtttatgaacaataatttagtttctcacctcatccaatttattgctaagagtttttttggtaaaattctgtcttggaaggcctactggggaaaaagtaagggattttaaacctctttagtgttgtggccatttcttaaaaatgagctaaaatgccctttttgaaagaaatatgattcagaagccatcagaggatcttaaatatggcggtgaggatggaacccattgctgcccacgtgctaggcaagctagcagacacgtgccagcagaccagaaagtgtagcgctgatgatcacagacgaaggacttacgtggtgctgccatccaagcccaatttctcaaactaactgaacatgcttctgttgccatgggtataatataacataggctgggtggttttttgttttgttttgttttttgcctaattttacatggtttatcctgtgaccttcacagcatcatcctacttcctttgcattaggccttgagtgtaaccagcccattgctctacccagtcggagaactgatggttttagtttggggttttttatgggttttgccctagtggttacaaaacaggttttttcttctccttagcactacatgctaagaacacatttgttaccatcccgcccgctctgggatttgtatggaagccagggtgttgagcatgccacttgagcactaagccatgaccttagcctcccacctgcttttgtacaaaagcgtagtttttactgatttgagatgcaccacagtgcacttgggtttgggaacacatttgtaggagtggttttgttgcaccaagtgatcatcaggcctgatttggatggcgcctggcttgaattttatgggatagttctagaggccctgcagcagcccacaccatcctgcccactgcttcaccgataagtccagaattcctcagaagtgatctcttgaaagtgttaaggtttgtggaaaatgtgaattgttttttttttttcccctacagaca

SEQ ID NO: 4 - DNA, 4000 bp, Cricetulus griseus
  source 1..4000: mol_type = genomic DNA
atatagtagccagttgctttctttctttttttattagtattatatttgggggttggagatggaggtcagaggacagttgacagttctccctttcagcgctgggtcctaggactcgaactcagggtatcaggcatgatggcaggtgcctttgcccagagtcatctcactggctctaagacagctggtttttaatggctatcagtacctttctttctttgagatatggtctcatcattttcttgcctggcttggagctcattatgtagacaaggctagccttgctctcaagagatctgcctgcttccgtctacccagccagagccgtgattaaaccccagatttactttcttgatggaaaaggttaaatgacttcacccgccccttccggtcatttgcctcatcgctgtggaatattactagacttctggcctacataaaaccctaaactcaccgtgctttggtggctcacacctttaatcccagcacttgggaggcagaggcaggcgatctcagtgagttcgaggccagccgggtctacagtacgagttccaggacagcctctaaaacaatacaaagaaacaccaaaacaaaaccctaaactctaaacacaaatacaggcctcaaaaatgcaggtaggtttgatgtagttcactaccagagggaaaagatatattaaatctttcaagaaaggcaccttaacggggaaaagtagtaaattcacgctgcggtggagctgggggagaaaggagggttctaaagggtagggtggagcagctaagtaaagggtgcagcctttacttagcacaagtgggaccctgggttcgatgccctgcacacaacaaccaaatgattaggtaatgttacggggaagttcactttcctttggctacctctgcgtgaggctctccgcagcaaggacaaaaggacagggtcaccttggcgggtggcacccgacagccaggaccaggatccgcgggggtgggggggggtgggggtggggggcacgcagcgcgcaggcgcggtgtcccacacccccctccccgcgccgcgttccacgcgagtgaggctcccacgctgcggcttaacgtttccacgccgctggggtctcccacacctcggggcggggccgggccgcgaaggtcaccaccaaggtcgagagccggacgtgctcgccgcctccaagccgagtgcgtgtgggactcggagtacgtgcggcgggccggagcccgcatgtcggctgcgtagcgacgccccgccctcacccagactccgcagaccctcagctcagcccccggctagcaacgggaggctcgcccagtaggccgaaaatgccacaggcccagccaaccaagtctacccccgcccccgggccatcgtcctcagactgtccgagccaggaggacacctcagtcacgctcttcttctggagtgacagcgccgggggccaatgcccggacggagaggacagagggcgggcccgaaacgccaagaatgggcgggccctcccgagctgctcacaaagtcggagtgggaggcgcttagaccagctcgggaaccggctcgtgcgcacgtccctgctaaacgctctccagggtgtgtataggaacctctgttcttttcctgctcgcccaccggagtgccaggtagggatcgggggcccctggggaacggttcgctcacgagctccgcgtggggggccccggtgggtgtgtgtgcgcccctccagcctgggcgcgtgcccggggactcgggaagcgttcggggcagcctcgtggagggacgtgggctcttggagggggctggggaggtgcagatccacctgttagcatccagacacaggcttgcagggcaactgggctcccaagcctacaaccgcaagtgcagaacagggtggatcgccgcccgggggggttagctaactggaggaaggctttttttttttttttttttttgagggggagaatgatttgacctaatgctcaggaaaaaccttcacaaaatggaagggcctgaaagaaggatgcccaagaggcggtccctcgtcatcgtccgcctccccccccccccccccgggctgctcgcagatcctgctagggctgtggctcatggaccgcaatctagcgtcactgggcgggagtggtccagcccatctctgccacggaatatactccggtgcttattctaggggaaattgcagcagaacccctggatagctggggagggcttaggcgacctcgccccagttaggcaagagttgcgggcttcctgagtggctgctagcaggccgagaaccgacttaggatgtgtttcaggaaatttcctgtcgcccctggcgtaagcagcgtggtccttttgctttcgtgggaggccagagccggcctgggcggatactttgacctctaggtccactattctgccccggctccggccttcagtccacttaaaagacctagagggtgagatttttatcctgggcaaagacagtgcagcccaacttagggatccgagtcagatgcatgctggaaggggagaaccaactcctacacgttagcctgacttcctagtgcgcgctggcacgtgggcgctcccccggcccaaatagatgaaaagaaaactaaagggccattgtgccagacaaggtgatgcgcacatataaacccggcacagggggcgctgcgacaggaggatcacttgagttcgggtcaacccggtatacataggacgtgggggtgggagaagacaaagaagtaaatggtatttaggcccagactgttatacaaaagtgtatttgaagtctacatagtaaatcattggtgttttaagatggaggttttttgtaacatagaggggtaaaaagtagatacttttcttgattagggtgtaaagatcctttgtctcacacaagacaaagcaacagaagaagctactcagttgaaacaaaaagatgcctttgcagcttcggcccttgccgtacgagacgtggagaacccagttagataaagatagtttatgaacaataatttagtttctcacctcatccaatttattgctaagagtttttttggtaaaattctgtcttggaaggcctactggggaaaaagtaagggattttaaacctctttagtgttgtggccatttcttaaaaatgagctaaaatgccctttttgaaagaaatatgattcagaagccatcagaggatcttaaatatggcggtgaggatggaacccattgctgcccacgtgctaggcaagctagcagacacgtgccagcagaccagaaagtgtagcgctgatgatcacagacgaaggacttacgtggtgctgccatccaagcccaatttctcaaactaactgaacatgcttctgttgccatgggtataatataacataggctgggtggttttttgttttgttttgttttttgcctaattttacatggtttatcctgtgaccttcacagcatcatcctacttcctttgcattaggccttgagtgtaaccagcccattgctctacccagtcggagaactgatggttttagtttggggttttttatgggttttgccctagtggttacaaaacaggttttttcttctccttagcactacatgctaagaacacatttgttaccatcccgcccgctctgggatttgtatggaagccagggtgttgagcatgccacttgagcactaagccatgaccttagcctcccacctgcttttgtacaaaagcgtagtttttactgatttgagatgcaccacagtgcacttgggtttgggaacacatttgtaggagtggttttgttgcaccaagtgatcatcaggcctgatttggatggcgcctggcttgaattttatgggatagttctagaggccctgcagcagcccacaccatcctgcccactgcttcaccgataagtccagaattcctcagaagtgatctcttgaaagtgttaaggtttgtggaaaatgtgaattgttttttttttttcccctacagaca

SEQ ID NO: 5 - DNA, 8450 bp, Homo sapiens
  source 1..8450: mol_type = genomic DNA
attttgcttgaaaggatagcatcaaggaagtgaaatgacaacccacagaatgagagataatttttgcaaatcatgtatctgataagggacctgtagtcagaatatgcaaagaacccttacaattcaataagacaacccaatttaaaaacaggcaaaggatgtgaataggcatttctccaaagatacggaaaaacggccaataagcacataaaaagatgctcaaaatcatttgccatttgggaaatgcaatcaaaaccacaatgaggtatcacttcacgcccattagggtggctatagatcagaaagtcagataacatgtgttggcaagcacatggaaacactgaagtccttacacactgctggtaggaatgtaaaatggtgcagccactgtggaaaacagttttccaatttctcaaaatgttaaacacagttatcatacacccaagcaattctactcttaggtatatacccaagagaaatgaaaacatatgtcttcaccagaacttgctgttcacagcagcattatgcataatagaccaaaagtggaaacaactcaactgcccatcaactggtgaatggataagtaaaatgtgatgtaaccagtcattggactgtcattcattaataaaaagaacaaggtactgattcatgttctaacatgagtgaatcttgaaaacactatgctaaattaaagaagccagtcacaaaaggccgtgtattgcatgattttatatatacatgaacttttatatatatataattatatatattatatataattttatatatataaatttctatatataaatatataaaatcatatatatgatatatattttttcatatacatcatatatatttacaaaaattatatatcatatatcatatgatatatgagatatatatcatgatatatatgatatatgatatatatcatatgagatatatgatatcatgagatatatgatatcatatgatatatatgatatagatatcatatgatatatatataatatatatatgatagatatattatatatgatagatatgatagatatcatattatatatgatagatatgatagatatcatattatatatgatagatatagatatcatattatatatgatagatatgatagatatcatattatatatgatagatatgatagatatcatattatatatgatagatatgatagatatcatattatatatgatagatatgatagatatcatattatatatgatagatatgatagatatcatattatatatgatagatatgatagatatcatattatatatgatagatatgatagatatcatattatatatgatagatatgatagatatcatattatatatgatagatatgatagatatcatattatatatgatagatatgatagatatcatattatatatgatagatatgatagatatcatattatatatgatatcatatatataccacatacatcatatatacatcatatatacatcatatatatcatacatatatatgaactttccagaataggtatatcaataaagacaggaagtatacaagtggttgccacagcctgagaggagcagggaatggtgagtgactgctaatggatatggcactttttttggggggtgatgaaaatgttctggtcagacaatggcaattacaaaactgtatacacacgaaaaaccaaagaatcacacactttaaaagggaggatttagctcggcatggtggcatgcgcctgtactcccagttactcgggaggctgaagcaggactgcttagagcccaggacttcaaggctgcagcgagctatgatcgctccactgcactccaacaaggatgacagtgcgagacccgttttctaaataataataataataataataataaataacccaaggtacccagttcacatgcaaaaccactggtaaacataaattatctccaagtaatctagaaagaaaatgagcacataagacgtcttctaaaaacacacatatatttctttacatgttacatttaacgtaaaaatcagctatgcagaagttacatgaacattttatgttggaaaggtaaatgactattattaatacagaatggttaagtacatttatgtttttatgtacaaacgcataaaaggaaaagcatccttaaaataaacaccatcaatggctcctcggtggtcacaaaacaaaatcctcacacctttgtcttccttcacaattgagctttatccaccttttcaggcttatctcccattattacctgacacaaacttgggtgggccagagtttccactgaccatcccccgactattcatccaacactatgttcactgcctcccattcctgaccatttgccttttgtcttcaactaattctggggacgttttgtccaaataaatgatccatattcttgaaggctggaatcaagtcctattacaaatatattttctcaccctctccagagcatagcaacccagcatctactggcctctcacagctctaaccatccacaaccctaagctggcttctcatcaaacgggtacttttcaccacccaaattcaattaattcactcttacaataatgaagaatagtcgcctacagcctaccttttccagccttgattcaatcatttatcaattttatcttcaaagtccctcacttcagggagatgatatatcagctttcacccagagtcctaaagaaaacagcactcttgccaatgacatagtgccacctagtggcaacataaggtaaatcacagtggcagtagaaggatctccacactacttttacaggaatgcactgcaggtaaaaaataagaagctacagtactgtttggcaggacaatttgtttcatacgtgcatactatcgccctgactaaattaactcgcaagtcttacaggtattatttgttttcagttccatgcacagattagccatttagtacttactaaatcaaactcaatttctgaagtgtcttacaccaatatattcatgcacatatggttaaaattttccttgaggatctatcatgtgagagtgtggcttattataacaagtaaacagaacaaataaatacaaaatgaaaagaaatcgtatgatttactcgcatataagggagcttgttgtggattaagtttcatgacccaggacactgaaacagaaatggaataaatgagaataaaattaaaagttgtcatcaaaaatatagaagccatctaaagacctaggtgtcaagcatagctctatgagtacaatcccgtgcctgagattaccatatgcccagctgtatgctatacactaagagatttaggaaggaagcggggtcagggattgaccccagactccatcttttcaagtggggaagaaagatcttccgattgaaaaataaaggcaaaaaaggcttcaccgtcacagaagtttcaacaaccaacaggatatttaaaacagttatcaaagcaaaaccattgtatgttcacttacatttttacatagtccctcaaactcacaaaatgctgtttactcagggacttcttccggtcttactagggagcctggaaagtgacgggaggattgcaagggaccactagaaccctcttcctcaattccccttctctgagaagggaggctacagcttgcctctctaaccactaaaaggcatgaccctcctcaaagttaatagccggattccctgatagatattttcactaaatgaattctcataaaactctcactaagatttagagaaggcttccagggttgaattcctgaacattaagaacagcatgttttttaaaagtttaacttggtgattggaccaggacttcatctaggctatgaatgctcagaatggtaggtcctttaccaaacagcttgagtttgtgtataaagtgatctcatcctcttaagagtcagagaaacagaaccaagcgacttcactataatttgatctgaggaagtttcttactcacaataggtaaatgaaggcacatactaaccagcaatataaacaacaatatcaagtgtcattcacacatgcaaaaaacagacaaaatcccaaactctgtgttctaacaaatcgcaaaaacctcactaacaataaattgaaatgaccaaatgtttggactgaaaagcaatgccttggtagcctagccatgcctaactcaaataacagaaccatctcgatgttaaaatcctcacagatcaagctgtgtatgtctcgggtcaagacttcgccaaaaagcagtgagcacacacttaagagggaaaaaatctacctcagcctcctaaatgcaatcatctctacacgagttgcaggccccaagcttcaacgtgttctgctggacaacgcagtagaaagctgacaagcaggtggccttcccacactgactgaaccacctccatgcccatgtccattcattttcttgcccaccccatgtgctataacagacctcctggctcagggcactctttccttcctgactgccttcacttaatgactttgtacttttaggtgcaaaaattatctgcagaaatccacactgaaaaccaagcttgagaaaggcagcaataaccaacatttttacaagaagaacaaggtcaatatcaagcccatcagattcaaatagcaagcatggatgaaaatgaaagattgaaaggcttgagtgccttcttaatgtattaaatatccatttaatttacaattaagctcactgtgctcactggccttttaatcagctttccaggtcctgctcagacttgcctaggacatgggaatgaaagaacctatacatttatggaccaatctaccttaactaacttgtcaagtgttcctgcatcaagcagaagaaacatcagtgaaactgatacaggaattaaccccttgttaatccataaaacttaaaggagcgggatccaatcttctggcttccctgggccacgctggaagaagaattgtcttgcgccacacataaaatacacgaacactaataatagctgctaagctttaaaaaaattgcaaaaaaggaaaatctcataattttttgtttgttgtgaggtggagcctcactctgtcacccaggccggagtgcagtggcaccatcttggctcactgcaacctctgcctcctgggttcaagccattctcctgcctcagcctcccgagtagctgggatgataggcgtgtgccaccatgcccagctaattttcgtatttttagtagagacggggtttcaccatgttggccaggctggtctcaaactcctgacctcaggtgatccacccacctcggcctcccaaagtgctgggattacaggtgtgagccaccgtgcccggccaatgttttaagaacgtttacgaatttgtattgggccacattcaaagccttcacaggctgcatgcagcctgcaggccgcggttggacaagcttggattagagaaatctacagagacaaactagtgacttagtagccctctgatagctcatgatttgcaagaaacttaggatgactatgtgtaaagaccacaaacatcaatttaactgaatggttcccgccacactggaatgaggaagctgagcaaactcagaggactctaagaaagggctgatgtcatctgaactgttcggaattataaactcctctaaacatgtttcaaagccagaacttgtaggagttgttctgatacacggattaaaagagggatgacaaagtgtctgtcccccacactggtcaaagggacaggtcattgttatgctggcaatgcaggctgctgaaaagaatgtatctgtcaaaagtaatcaaagtaatgaccccagaaggctccagaaacagactggtaaattcaggttgctttcagacttccacaatgctggcacacaaggggaaagacaaaactaacatttacagagcattatatttgatattacatttaatccccattaaaaagatactatttcccgtttcactagtgaaaaagttgatctttcaaaggttaaattatttaacaccaaggtcaaagggtaagttggagagaccagattcaaacccagtctgacattaaaacatgtgttttccccccacatcgtctcctgctaataacctcaaatctaaaaactgacttgccctacaccttgagccccatcctacaaactctccctgacgttattaattcagctgtcactgtgcacctacaacgtgccagacaccatactcctcaacactctgtaggcacagaaggaacagataaaaatccctaccttcatagatattattctaggggtaacacaggtaaataaaacattaaaatagttttcacatagtagcaaattccatatagcaaaataaaacagaagaaggaatagcaaatgagggagatgccctcttaaacatggtgctgagggaaggcctccctgagaaagatatcatttaccccaaaaataaaaaagcaagtaatagaaaaaacaggtaaaaggtgttctagacacttaaacctgccacattgagaactcagggttctgatgcaaaacctcgctgcatagaatgcattaacttatttttatacatttaaacaaacaaactctacttaagaactgtgttctaaaggaaggagcatattacaggaaggcaatttttggtcagagtagacacacttaaaaactaaacctattgaaagaccaagaacaactgaaagtctttgctttgtcagatttttgaccaaaaggaaaattaaagaaacacaccgtgcccatccaatgatttcaccaaggaattttaagagagaaaatcctacttcttcctcacccagtagccagtgaaatgactgagcaaattcacaagttcactggggctgctttcatgtaacacagggacaacacatgacagacacagtggaaccctacaggttgcctagtatttgaaagactgtgaagaggaggagatgtcaaaattcaaagtcttaaatgatgtagttttaagtatgttcagcaatttcaccactcagtagtaaagccagctacagttgaaagcaatcagaaatttgaggggtgtgaaataagcagaagcacagaagttaaggatttgtattcttcccacattttccactttattttatactgctgagaaaaaacaaatttaatagttttctgctgtataagagagacacattcactttatgtcacagtaagagtcactcaattttaatacaactatctcaatgtataaattaacattctcccccctgcccacacatagtaagtctcttatgatgttgctgattagagaagcaaaagttgccgctacaattctcttcctgcattttaatataaacaatcatcagtcttttcttcatagagtgcagtgtgggcactatcatcagaatgtaccagcactgggtgtgcaaagtttacaaagattagcaagagcaaaagtgttgagatttttgaaattcatgctgctgcaaagaagtatgtaaaaactcactcaccatagaggaccacacagaaactcaggcatgaagttatatggctgtgtgagtggtttgggagaaggaacggaaagcacttccaccaacctatatgcctgagcaaattaatgcaaaacctcagaagctacaaaaaagtttatctacctaaattaaaattggtgtccacagcagtagccagcaaaatgcctgcgaagcgcaaagtggtaaatattttagggtctgtaggtcatatggtctctgttaaacaatatgtaaatgaatgggtgtggctgtgttccaataaaacttcatttataaaaagaggcagcatggtacatccagtcagcaagctataatgtaccaacccccggtctaacactaaccaaatacctcttaataagccaaagaaactgtgtcctcttaggccggaagcggtggctcacacctataatcccagcattttgggaggccgaggcggggagatcacctgaggtcaggagtttgagaccatcctggccaacatggtgaaaccctatttctactaaaaatacaaaaattagccaggcgtgctggcgggcgcctgtaatgccaactactggggaggctgaagcacgagaatcgcttgaacccaggaggcagaggttgcagcgagcctagatcacgccattgcactccagcctgggcaacaagagagaaactccgtctcaaaaaaaaaaaaggaaataaaagtatacaaagtgaaaacaaagaaattaaactgcccttatttgccagtgacattactgtctatgcacaaaattccaaaaatctacaaaaaagcttctagtactaaaaatgagtttagcaaggttgtagaatccaaggtcagcatataacataaaatcaccttcctatatactagcaatcaccaactggaaattgagaagtatcattcacaacagtaccacaaacatgaaataaatgtg

SEQ ID NO: 6 - DNA, 8420 bp, Homo sapiens
  source 1..8420: mol_type = genomic DNA
tcttagtatggtaaaccttttgaagtagattcaaatgagaatgggaagagagaaaagggagagaagcaacataagaaatctcttttaaggaattttatatagagagaaacagaggaatcagttgatagttggaaattattttaaagaaaatgggttattttaaagaaaaaaggtattacaacatgtttgcactattgtgggaataatcaagttgagacagaaaattattttttaaggaagagtctaattgctgaagtgaaagagaatgaatgagaccctgtgcataagtgtgatcagataggagcatgtacagctcaagtaagaacaggaagaaagagacaataaacatgtacagataggatgggctggtcgatgtggtggtgaaaagacatgcgagttattactgattacttctatttccccagtgaaataggaagccaggttcataaaccaaaatgaagaggagcgaggcagtattggaagttcaggaaaagtaataggtgtaaaaatatgtaaagtagaattaccagggagtatgaagatacatttccaattaaggatgaagaatttaaagtgaggccagccaatacccctgctttgcttcagctacatcagctgcataggttcaggcacagaatacatggaacattgtatttaaatagggcctggattttacaaaagtaacacaatgaagaagagagatgcaaggctatttgagggtgtttgtgggagagattgtaaaatattagctaagtaagaaggggactgcaaattttagtggtataaaggaatgaggaaaagtgtaaatacagtggggtcaaagaatgtttggagccaaggcactagaggcaattagctgaaaatgtaggtgattattggtgagtgacatggtttaaatgaaaagtatagaagggtacaattatccatcatgaaaagttctagggtacaactaagatctgagtagctgaagtagaatgaaagtagaatggacctttccatatccagccaggttcagtgacagaaggttaggaaacaaattataaaccacttgagagaacatatcccctaagttgtttttgctatttttctttcagcatatatttgttggaatgccaactatgttcagttcaattaatatgggcttcttaaataagggctccagcactggataatcctgccatttattttgatacattccatcctgctgctcagatctattggcatctacaggatgtcttttgagaagatgggcattcacatccctatgtcctagcaaatttccaactcagaaaaccacattaggcttctctatatatcttccaactatttcaatggaaaatacaattctctgatttcttcctatgatatttatcaaagagaatggtgcctgccagttctagggtgggggaactcaatacaaatcaccaacctttagatgacaccctgtcttcaaagtgctttcaaagtctggcagaaaaaaagtacccagtggctataagaccacccaggagttcagtcatgcattctaagtagcagatcactggaatgtaattggctagtgagttcattttactcttctcttcttggtcacatgttaccgcccttgtaccctgcacgttctctttcccagacttacaaagcatgttctcttgaattcgttctctttttaaattcacacagtcttaatgattcttctttcacaagagtctttcactcttacaattcagttcaagtcatccacatgcttattatgagcaagggtctgggacttaggggaaaagggaataaaaagatgaatgaaatgtgatccctgcagtccaagagcttgctgtgaaaaaggaagtttggcttacattgcctccctaatcccttggctaggccagaacagaatattgtctaaaacctcctcacgtcagcagtcctctggggtggtgactggaagtagaatttaaacaaaaatataattgacacataataattgtgcatacttatagggtacaatctgatgtttcgatatgtgtttaaatgggtgcattgtgtaatgatcaaattgaggtaatttatccaccaccttgaagagagatttttcaatattctcattgcgaagaagcaggaatttttagcagacaactgagatgcttcttgttcacactaagtcattctgacgatggatttacataacttgttgttttttttgtgtgtgtgtttttgagacagagtcttactttgtcgactaggctgaagtgcagtggcacaatctcggctcactgcaacctccacctcccgggttcaaacgattctcctgcctcagcctcctgagtagctgggattacaggtgcatgcaactaggcctggctaatttttatatttttaatacagatgggatttcaccatgttggccctgctggtgtcaaattcgtggcctcaagtgatctaccagctgcggcctcccaaagtgcagggattacaggtgtgagacaccaagcctggtacatttacatttcttatctggatctttcctttagtaagtgctaaggaatcctacttcccccaatattttttcctatttcaatgttttagcatgtatcatgttactactttgcagacatttgattttcccctttgtttactgtaaagtatatttttatagcctttgtaatagaagtattctaaaatctgcctgcaacctatctttctgactctgcattttagggaataattctctgttgtggaatgaaaaaaaaaacagagcctgtggagtcagagatctcatttcaaattatagttatccctaggaataaatctgagtgacaggtagtatagtataataataagtataaagctatggttaaggaaaactcaacaaccttatctgtaaattgggatgacaacagcctacgtcaaaaaaatgtgaaggtaaatgagataatgtaaggctgatacttagtaagcaatttaaaaacacccaaaaaactattgccatgattactctacttactctatttctctatgctccaggcaaatgaactactaatgacccaggggtccttccccattctcttcttcacaaggaaatattctctctctgtgtgctgtttattaaaatctactgccccttttagaagcctttccagatcatcccatggccaagaacgatcgctgcttcctcttctttacatacagatgtttttctcctgcttgacaattatttttgtgcaattattttccttttgattgtgtttttaatgtcccccccaccccacaattttccagactgtttgctccacgagagaggagaccatcatctctgtgctcaccgttgtatgaccagtatcctgaggagtggctgttacataattacatcaggcactcaataaaaatttgatgaataaacactggattttaaggcaggtatcatatcttacatagcatatcatatcttacattttatgtccctcacataaataccacagagtgaagtatatgacagataaggtcatttctcttgataagtacatagtccagtctgaaacagatatgccaaaaaaaaacaaaactggagtaaacaagatgaattgttttaatagaggcactgtattagtttcctaggactgccagaacaaatcacctcaaacttagtggctgaaaacaacaaaaatttattgtctcacagttatagatgttagaagtataaaattaaggtgtcagtgggattggttccttctgggggctgtggaagagaatctgtcccaagccttcacactgtaaagtacagtactggagggataggacttcaacttgctctatctcagatagagaggagccatttgttgtgaattgagaagaggggtatgttgaatccataataagcacataaaaacttggctggttcataggagaagtaacatgtttccagctctagtaaaaaacaaattgaagtggcctataaaaaggtacagagtacgacagaatgaaaaataaatgaacaagaatacagagaggatgtggtaaattatcatgtttccctaatatgttattggacactaaatggtattagaattatttatcaataataattctaaactgttgcaattgaaagaatatattaagtggtgttatatgagaagtgccagggcattctcatttctgtccaatgggagaaacattttcgtttgagacctccgtgaataatacagtcttttagttaggagagctgcattttgagtggtgcaggcagaatggcgatctctcacccacacaaacactaagatagagagagacagagacagagacagagacagcagagagagacagagaaaggaagtacaggtactcagatagagataagccatttcttgacattaagaaataaagtagaatccattggagggaaataaaactgcctcaggaacagagttaattcacatacacatgcaggtaaacacacactgcttgatacttactgtggactttgaaaattatgaatgtgtgtgtgtgtgtgtgtgtacattcagccctccatatccatggattttgcattcacagattcaaccaaccatgaattaaaaacatttggaaataacaaacattaaaatataacaatacaacaataaaaataatacaaataaaaaatatagtgtaacaactgtttacatagcatgtatgttgtattaagtagtataaatctagagattacttaatgtataccagaggatgcataggctatatgcaaatactatgccactttaaactgataagaacagatactaaacttcatcttagccaaaagtcagagaaacaatataactatgccattttacataagggacttgagctgagcatcctcagatttcagtatctttggagttcctggaaacaattccttgttttatatatatatatgtgtgtgtatatatatatatatatatacacacatatatatatatatatatatatgatagctactgagtgacaggtgatattataccataccacttgtcactcagtagctgtatatgcatatgtatatatatacatatacatatatgtgtgtatgtgtatgtgtgtgtgtgtgtgtgtgtgtgtgtatgctgtctttcctcggtatcacagggaattggagatatatatattcttttcagtacaaaaaaaattgaacacagatgggtatggtaccagaacagaaggtaaagacacatgaaaaaaatttgcaacaacatgaatggaactggagatcattatttgaggagaaataatccaggcacagaaaaacaagcattttattattttaggtgaaagacaaacattttattttaggtgaaataatccaggcacagaaagacaaacattgcatgttctcatttatttgtgggatgtaaaaatcaaaacaatagaacgtatggaggtagacagcagaaggatagttaccaaaggctgcaaagggtagtgtaggctttgagggtgaggtggggatggttattgggtacaaaaaatagttagaaagaataaataatatctagtatttaatagcacaacaggttgactatagtcaaaataacataattgtacaatttaaatatgaaattaaatatatatacaagactagaacaccaagttgaatgactccagcttgcgaaacccacattgatcaccatgcttgccccaagggaagctgtacaatgtctggctcgtccagaaccccatcatttatcactagcaatctattgtccataatcatgtttaaattaatagcattttaaaggtacaaatattttttaaaaaacaaataattatttaattcgccttttaaaagctttttaaaaacgtttttaaaaacttttttaaagtcctgaggactattttctttaaagtgctcagttacagagctccatatattgggctatgatagccttacctgattcttgccaagaatctagtgcccagaaaatgcaaatacaaagtaagcaactgaaaaataaacaaataagttggaggtatgctacctgttgaaatatgacctagcgcaaacacctatgccacttgcttatgaaatcatataggttttcggtgtgcagttttgactgaatgagggagtttacgctggaccacaagggggcccctctgtcaataacgtactccatttgtgtattaagtcaaaaatgaaatggaagagaaaagaaacatcgatgaccccaagtctctttaattgaatggaggtaaaagggaaacaacgaatgagaaaagtactctgcccttttaagaatcttgcattcacattcctgatgaagttatttttcctcctctcactgattcccatttcactctattacatagcaccgtgttccccaggagctcctgaatgaaggacatcactcagctgtgttaagtatctggaacaataaatatactagtttcaatgtctaggctatgggtattcctttttactgaaggtatgacatatagctgcccaggcctgactaaattaatagtaataataattaataatggcaaatttttattctattaagttacttggcttgacttgtagaaatagcaacattcatctgaaatgccccctcctacacttatgtctaaggacaaatcccacatacaccacagataacttcattttacatgttttattctgttaccaaactaaatttttatcatatagtctgttgctcactgaactcttcagtaattctcaacataccatgtaaagcattaagcacagttccaacacagagcaaatgagcaataactgttagttattataacattattatgtgttttcagtgcattaaaccactggtctgatacctagcccaacattctattaaaccacataatccagttgaataatatatgataatataataaaatggcgataagtgctaaatatccagatagaaacacagatggaatcagacagctttcccaagaaatagagaaaatagtagataggcgatctaggcctaagcactctaagcagaagctaagttatcacaggatatcttggcaatctgtggcacgtgaacccttttcttctggagtctggaactatgttgcaactctcactttctccctatctagagactcagtttgttcccttgtgattatcagcagttgagaaatccttagaccttctgaaaggactactttttaaatttatatatataatatttaaaatacatatctttatatataatatatatttaaatatataatatttaaattaatatatatttaaatatataatatttaaattaatatatatttaaataaataaatttatatttaaatatataataattaaaatatatttttaatgaacagagagtaaaggattattttgaagagaaactcctggttcccacttaaaatcctttcttgtttccaagtttttcaaatggagccctctttaccagcttgccccctcagagataagctgttcccctacttattcagatctgagatctgaaaacattccttttcctgtgagttcagctaggacaaagatggagctttttgataaaatttggcaaacacattttttaaagatgaaaatttttaaaaattgaaaaaaaaacatttatagaaagagacttctaatccaaatttaacttctcaaactatgttttgaccggctagcataatgtttcagtctttctggagaatgccccttgaaactgttttcttctacacaacttcctcctttcctttgactttcctgctctggaagggaagaacaggaagaggacagatcaaattactcaagaggaaggacaagaaataaggaaccaaattatcaacaattggagaaagaaagctgatgtcagtatcatttcatatatgattatgtcagagtcaggtggataagccaatcctgttgaatagcatacttttcctgctactcctgaagggtaaagaggtctttctcttacaaagccgtcctagctagtaatcttacaggtgcaaaaagcttgttttcatgttatttcttagtaactcaaaatacctctaaagttatacatattatgaaagtactacagtcacagtgctgagaaaaggagtaaataagacaatgtatataaaaacacttggctcagcccctggctctgtggttgataaatattaagttagtattcattattattataatttccaaagagtccattaaaagatatagaagaagggaggcagcaataacactaagagaaaattccattatctccaactatttatcctctagcccaaaataattgccattagaaagagcaactttaacaaaaattttaagttgcaatagatgttcaactttaaatccatcccagaaaaatttctaaccaaaggagcatagaagatttgatcttattttctaagtagtatagacttaattgtgagaacaaaataaaaacttg

SEQ ID NO: 7 - DNA, 8475 bp, Homo sapiens
  source 1..8475: mol_type = genomic DNA
gcataacttgtaagaaatggagtgaggtctcagttcaaactggcttctgtatgacttcaaagccaaagtcagcaacttagaaggcaaaaattataatttagttggcaaatacgagaaaaggtcagaaacacatgaaatgaagctcaataggaacacttacagggtagcagggtagtagcctagggaaaaaagtcagacactaaaattgtttaaataggtaagttcaagggacaggtaaagaccttagtgggtaagaagccaatcagcagacgaactgcaagcaagcactgtctctctttcccttctgtctcctcttgtagtaactgaccacaattaaggctgcctaggggaataatgaagtaatcctcctattatcagcaatggtctgatccagtgccaggcaccacagacaacttggtgttcagagaagatccttcaagatgaacaaagggtcaaaataaaaaattctagaagagagaagactgatcacaatttaatgtaaggcttggaaggaactgatctctaccttccttaacatctcaagaacttcctcagattcattggatgttgagtgtgtgtgagtctagtagaaaaatgaatttttgtttcttaacttggatatgtgattaggatgttaataattaagtctgggctaatattgaaggtatcttatgatgggcttcttaaagcattgatcacaaagactgcatgttcataaactgagctgcacttgttaggattctagatgtttgaaatttcttgtgttattttggtctcagatttctagacaaattttctcaaattcctatttcactttttgacatatcatgagtgactcaaatgtttgcccttgagtcggaaaacacccagcattaggaataggcacataaacataatacttcaagcttcagatttaagctcaattataaagtgtttaaaggctgtgctgatagttcttctgagtagaattcctacaactatgggtttgtctataataaaatgttcactctatattgaacgccttatttaaaactcgaaatgtgtaagtagtaataaagaaaatatgtcctcctgtaaccaaagctaggaccgattacatgttcacttgactgacagatacaatcacctatattaggagcaatcagcacttccttacaaactaacaacttgagatgtagtgttcccattggctatgaagattttctttatttactcagaatagtctgtaggatctgccagctgcccctgattataccagctgcacccaatgatcacagtgaacattattttacattctaaataactggtgcaaggtgagccatggttttctgagtttcctatcacctttgtgtttcaggtcctcaaatgttaatttgtaaagctgctgtttcaggcaaaactaacaaaattagcatctaatcaataaccatactatgtccacccatatcctataacacagaagtaggggaagagtgagaaaggtggaagtggagaaatagaggcccaaaaagaaagttttatcacaggaatatctagatgtcttctgggattgtctgttaaagagctgtgacactcatataaatgcagaattactctctttcttccttgttggttagaaggccaagggtgccatggtaatactaccaaacatatatcaaagcttggcaggaaaaatggtaccttcagaaattttataatctgatatcaaataggtcaagaaatataataaaactagtttctttggtttccttagaaacctggaaaactttaaattagaaacttagaaagctttaaatcagactttgtagttaaaaaaggaaattttagttccttccagcattagaattccgtgattctctgactctgagcctggattaaatctagcccagctgagtggaaacttaagtaactagctggttgcctttagtgatcttccactttatggctgcttccgcctaagaagttcatcatcgtgacttactttctttggggcaaagtcgtgactaactttctttggggcaaagttggaaagcagaggtcaaagtcaatcagaaatgggacaaactcacttcctactgcctggtgaaggggccattttcagtagccccttttcaagattagtttcattcaagatttgataagctgttttgactttactatagatcttattatccatgtcagttaagtttatgcttccactaaatctatctgaattcaaaaggtaaaaagctaatgctcagtcttatcagatttatcttatttattaatagaatgtggatttttttaagcatataacaataatagtaatgataggaccataaatgtggatggctctttacaagtcactaacattacataaattcctcaacaacacactctgaggccataacaaacttttagaaataacacaattggctacggaactccagccatctagcttcatgggctcccactttaatttcaaaacaacagaactgtgcacattcatttacatgattagggcagagcttaactgtatctcatgtagcacctacatcattcttcagacaaacttattgccttttacagacaagaaaactggggctcaaaaaaggacttgcttataactggctaataaagaggaactctgggttcaaagtgagtccaattctttcttccacccacagcttctgctaaagtcattacagaaatgcatagagcagttcttccacgttattgcttaggtttctaaagagcagtgacctaatacaacatgctctataatttattactgatttaactatttcactaaggattcacttttaacttttaacttgtaaatatgtctaataaacaccactgaaatagcaacctctttcttcatggccttgtggttgtaaagcaagctagtaatatatgtctgtggatttgtgctaataaagttctatacacctcattaattccacaaatcctactgggtatttcttatctgccagatcctacgctaggtactggatacacagtactgaacaaaatgggtacaaatgagcctcacagagcttgtttcattgaaaagcagagagatacacactaatcaacaaattaatagtaacacactacgatgtgttttgaaggaaaattagagcatcaaagagacggtgttagcaggtggaggggagctcttttagatggagaatgagaatgcctccctaaagacatgggaataaattgagatcacaaaaaatgagaaatagccagccttgagaagagcagaaggaagaacattcaaaggaaaagaaagtgcatactggaaagcctgaacactagagtttggtgtatgtaaggagctgagcaatggtcacttgtgtgataagatgtgtggatgtggggtggggggcaggggtgagtcccacgcagctcttaagtgtgtcctcagactcctgtggtttccatcagccacaacctgaataactgtgtggtaatccaaaaatgattacagattaaacatataaaaatatcattacacccatagtacctaagccaaggacacagtattctatcttttcaatgaagatctgcatgaagtaaaattattatatataattttaggtattgatatagatacatcagtggatagatatagatatgtgtctctggtatagaaaaaagttttaaagggatattaaaagttcttatcttgcagggttgaagattgtggcaactttcatttctttttaattttaagaaaaaagtggtattatgggggattagcatgtttgtgggtatatgtatatttttaattaaaaaataaacaacaaaatgaaaacgtttttcttctatgaaagcctaataagaagaaatttcagctgttttaacttagggagctaaaaacatcaaatccaagaatgttctctggaactgagctcaatacatttttatttgagtaagaattggatacatttccatccccttggggctccagtctgtcaatattttacttttcagcgataaaaagacacatgtagataatcacagtgacctcagtaactttccttctcttatttaagtttattttatttctatcgtagttttccctgttaaagattttttctttttgcttacatatataattttagagaataacaatgcacacacaaaaaattcctcttgttctgctagacctggactttttctctaatatatatctccattttttgtcttttttcagacgtattttggaagcaaaggagagaattgctatatagctgacttcctcttctcatcaacagtgttttaacagtttttaagcaaaagtcagctttgtttatctaagattttttttgctggcatttaacctacccctgcctcccctttcccaagtccacttcagccaacctctcattcgacaggtaccaccctctaacataactgaaataatgtctaccattactggatcttgctagcaaagaatctcaaattttcccacttggttgtaaattattttgtaatctctagtgtttaaggtgcgcttgtcctatctaatcccctccctggcaggacaccttacagaacctaccccttacactagtcattaagcaccatcagggacggatggctgtgtcactggtctgtttggtattccctactgatcctaccatgtggtgattatctatgacttccctaatccctggctgccttagctgggactggctgacatgcttctcaggttgccgctggctttacagtcctttactgcccatgccactttggagataggcagggctagtacttttctatataagcccccaaacttgactttgtgtttcacagtaggtgaaaaagttgggtctcttttcttttacttttctttccacaagatgataaagctaggggaagcctgtggacatggtttatttctgcaactgcaatgattgattggtgcttcctgctgcttacttcctaaactttgtgctcagtgtcagatccctagcagtttctatcccctgctctgctaaaaaagaatggatgttgactctcaggccctagttctttttaattaaattgtatttttgttatcattattattattattattttgagatggggtcttactctgtcgcccaggctgaagtgcagtggtgcaatcacagctcactgttttagcctcctgagtagctgggactacaagcgtcatgccaccatgcttctttttaattttttaaaatggttttctgccttcaattctaagcacttctcaattgtaaccaagagataatactttttatgaattcttaaagttatcaacagatactcaaagttttagcaaagtctaaatgatattaagcttgtccttattgcccaagtgacttcaatgactatttgttaattgcaaccaagggtcattttttaaatgaatatatattattattatatatataatattaaggtcctcaaatacctaaaagtttagcaaaatctaaataatattgtgcatattcttttattactgtattagtccgttttcatgttgctgataaagacatacccaagactgggcaatttacaaaagaaagaggttcactggactcacagttccacgtggctggggaggcctcacaatcacggcagcttacgggattgttgagaaatgacacttctcaagctggggctaaactatctctgtggtagttgttctgattcaagtattgaattggttttttttgttttttttgagatggagtttcgttcttgttgcccaggctggagtgcaatggcacgatctcagctcaccgcaacctctgcctcccgggttcaagtgattctcctgcttcagcctcccaagtagctgggactacaggcatgagccaccacacccagctaattttgtatttttagtagagacatggtttctccatgttggtcaggctggtctcaaactcccaacctcaggtgatccacctgccttggcctcctaaagtgctgggattacaggcataagccaccgtgcccggctggagcattggtatataaaagctgcctaggtaactctaacctttggccccatacatctgaaggatacctacaatgcacctgaaaaatgcaactgaaacagtagttccctgggaccacacactcagaaagggggtgtatcaggagatctagggaccaggagggtggaagacctaaggcagcactacagatgatggagaaaaacccactggggaggggcgatcctaaccttgagaatcactgagatcatgcagaagtatttgatcctacagcattaatattgtattgtattgtattagtatatatatatagtgtatatatatagtattagtatatatattgtattgtattagcatatatatactaattgtattgtattgtatttatatatatagtattgtattagtatatatatacagtatatatgtatatatactaatacaatgtactaatacaatacaataccatatatatatacactaacacaatacaattagtatatatatatatatatatactaatacaatacaatactatatatatactaatacaatatatacatatatactcaccaagacatattagtggtctgatgtctggctgccacactcatcttctaccttcagctctgctctaccaaatatcatttgtttctgggatctttgcagtccaaggaacttcatccttgatatcccaccccttactaacttttttttttttttttttttttgagacggagtctcgctgtgtcacccaggctggagtgcagtggtgtgatctcggctcactgcaagctccacctcctgggatcacaccattctcctgcctcagcctcccaagtagctgggactacaggtgcccgccaccacaccaggctaatgttttaccgtgttagcaaggatggtctcgatctcctgacctcatgatccatccgccttggcctcctaaagtgctgggattacaggcataagccaccgcacccggccaccccttactaatttttagtaacgtccaaggattaaaggaaatttgccttacctatttaacaggaatcaacagggttaatctcactccctttctaaaaataatttataaacattgcagacaatctcatctatccctgtctaaactgtgtggaattactgccatttaatgtaatcagtctactcatttagtttgcctaaggaatttttgaaaaaacagttaaatgaatgacttaatggaataaccaggaagttgaagtctccaatagtaagaatgaactcttgctctctggataatcaaatgggtccttcctccttcaggtagatcatgccatttcctcacttacactgaacaggtaaacaacataattactgacttcaacttctagttaattccttcttttatcactgagtatcctttggctgggagttttgttggctatgctgccattttttctagttatcacagtcctataacataccaatccttcaatataactcatctttaaattgtggttttaccttctcaagaagttattaattatgccagtgctaaatcttctaaaatgattgttgacttgttgattagcccccatgcaattcccctctcccgtccctcagcacgtaaggaatggccctttgcttacttccacagatccttaaatctaccagttagaagctaatagcctacctctctaccaggaaggaactgtgggctggaacataatacatgttgacttataatttcttagaaaattgtgtgagaaacatcaaactcctgattccaggatatgccaaagacacatcattaaaaagcaaaacaaaacaaaacaaacctcatttgacgttgctagtagtggcatatttcatcaagatcagctcaaataaatagaagtgagattttcacacaaattagactgtagtgcttttttttttaacttatctttaccatatgatttttaacggtaaaaaaaatcgtttgagatattagatgtataatatttatcatccaattacttcattagttcaatcttttttcaatggcgctcctgcatctgagaataaggtcagaaaatttcatgttctgatttcatgctgattttcagaagaaaaatgttagttttgtatagaataacccatcctaagaaatacatttcttattatatttcttatcttatatttcttaggacaatgagctattcaaagggtgatgataaccagcaccatcagtcagcattatctaagaataagaatctgtgtttctacatacagacctcctaaaaaggaacctacacttaacaggattccccaggcaatttggatgcacattaaagcttgagcaacactgcattagaaagttagttttccatcacaaaaacagtaacaaaaggaatataaagtaagttactttaataatataagaagaggggcaggccgggcgcagtggctcacgcctgtaatcccagcactttgggaggctgaggcgggtggatcacctgaggtc

SEQ ID NO: 8 - DNA, 28 bp, synthetic construct
  misc_feature 1..28: note = Primer K24
  source 1..28: mol_type = other DNA
ttcgcggccgcggcacgcagcgcgcagg

SEQ ID NO: 9 - DNA, 34 bp, synthetic construct
  misc_feature 1..34: note = Primer K25
  source 1..34: mol_type = other DNA
ttcactagttgtctgtaggggaaaaaaaaaaaac

SEQ ID NO: 10 - DNA, 5000 bp, Cricetulus griseus
  source 1..5000: mol_type = genomic DNA
gttctttagacgtggttactcatttcctctcccggtgcctttgatctgccactgccatacaatcgcccaaccagcgcctgcaagtgagaaaagacgtataaatgcctgtgacaaggcaaacagccctgtgctggcttcagacaaatgtgagcagggcctgtaacagcctggagagccttggcaacagggcatgtggctgcttgtgaattctgagacatcctggaatcttgcaaaggcagctgcttgataccatgttgctttagattccggcctgagacacctggtctattggaataagagttatcttactctatctttatctctccaaccattttagtgtaaaacaaagaggctgtctggagccctctcagggccatagtcttggaatcacatggaaaacagagctcagagtgtcccacttcttacaaggtttggcaaagggagagttgttgcttcagctgctgagtcgtgagactgcagaatattccgttcatgcagccaacacacatcagcatattattggtgaaatcagactgcttgaaatccctaacattcgttaatgaatcattttacaatttccttgttgcttctttgttgaatttaatcccaaagatcttgcttcttcatctatggaaacttaacaccttggactcaataagccttcagtgttacccaaggcctcggaaaccttggtcaggaactgcctggagcaaaatgctaggggttaagagagaaatgcaacttcctgtagctgactagatgatagaataaccaaagcaaaaaaacatatttcaatctctctatgaaagacgatatggaaaatatagaaacaagagacattggcttccagacttacagcccagaagaaacagaaaatacaaccggaagagaggtgctgacttcagccctcccatgaagaaatatgtgcattccagagacttgcagattcttgtagtgtttgagacaggatcgtctcccttggtagcccaagcttgcctcaatatagtagccagttgctttctttctttttttattagtattatatttgggggttggagatggaggtcagaggacagttgacagttctccctttcagcgctgggtcctaggactcgaactcagggtatcaggcatgatggcaggtgcctttgcccagagtcatctcactggctctaagacagctggtttttaatggctatcagtacctttctttctttgagatatggtctcatcattttcttgcctggcttggagctcattatgtagacaaggctagccttgctctcaagagatctgcctgcttccgtctacccagccagagccgtgattaaaccccagatttactttcttgatggaaaaggttaaatgacttcacccgccccttccggtcatttgcctcatcgctgtggaatattactagacttctggcctacataaaaccctaaactcaccgtgctttggtggctcacacctttaatcccagcacttgggaggcagaggcaggcgatctcagtgagttcgaggccagccgggtctacagtacgagttccaggacagcctctaaaacaatacaaagaaacaccaaaacaaaaccctaaactctaaacacaaatacaggcctcaaaaatgcaggtaggtttgatgtagttcactaccagagggaaaagatatattaaatctttcaagaaaggcaccttaacggggaaaagtagtaaattcacgctgcggtggagctgggggagaaaggagggttctaaagggtagggtggagcagctaagtaaagggtgcagcctttacttagcacaagtgggaccctgggttcgatgccctgcacacaacaaccaaatgattaggtaatgttacggggaagttcactttcctttggctacctctgcgtgaggctctccgcagcaaggacaaaaggacagggtcaccttggcgggtggcacccgacagccaggaccaggatccgcgggggtgggggggggtgggggtggggggcacgcagcgcgcaggcgcggtgtcccacacccccctccccgcgccgcgttccacgcgagtgaggctcccacgctgcggcttaacgtttccacgccgctggggtctcccacacctcggggcggggccgggccgcgaaggtcaccaccaaggtcgagagccggacgtgctcgccgcctccaagccgagtgcgtgtgggactcggagtacgtgcggcgggccggagcccgcatgtcggctgcgtagcgacgccccgccctcacccagactccgcagaccctcagctcagcccccggctagcaacgggaggctcgcccagtaggccgaaaatgccacaggcccagccaaccaagtctacccccgcccccgggccatcgtcctcagactgtccgagccaggaggacacctcagtcacgctcttcttctggagtgacagcgccgggggccaatgcccggacggagaggacagagggcgggcccgaaacgccaagaatgggcgggccctcccgagctgctcacaaagtcggagtgggaggcgcttagaccagctcgggaaccggctcgtgcgcacgtccctgctaaacgctctccagggtgtgtataggaacctctgttcttttcctgctcgcccaccggagtgccaggtagggatcgggggcccctggggaacggttcgctcacgagctccgcgtggggggccccggtgggtgtgtgtgcgcccctccagcctgggcgcgtgcccggggactcgggaagcgttcggggcagcctcgtggagggacgtgggctcttggagggggctggggaggtgcagatccacctgttagcatccagacacaggcttgcagggcaactgggctcccaagcctacaaccgcaagtgcagaacagggtggatcgccgcccgggggggttagctaactggaggaaggctttttttttttttttttttttgagggggagaatgatttgacctaatgctcaggaaaaaccttcacaaaatggaagggcctgaaagaaggatgcccaagaggcggtccctcgtcatcgtccgcctccccccccccccccccgggctgctcgcagatcctgctagggctgtggctcatggaccgcaatctagcgtcactgggcgggagtggtccagcccatctctgccacggaatatactccggtgcttattctaggggaaattgcagcagaacccctggatagctggggagggcttaggcgacctcgccccagttaggcaagagttgcgggcttcctgagtggctgctagcaggccgagaaccgacttaggatgtgtttcaggaaatttcctgtcgcccctggcgtaagcagcgtggtccttttgctttcgtgggaggccagagccggcctgggcggatactttgacctctaggtccactattctgccccggctccggccttcagtccacttaaaagacctagagggtgagatttttatcctgggcaaagacagtgcagcccaacttagggatccgagtcagatgcatgctggaaggggagaaccaactcctacacgttagcctgacttcctagtgcgcgctggcacgtgggcgctcccccggcccaaatagatgaaaagaaaactaaagggccattgtgccagacaaggtgatgcgcacatataaacccggcacagggggcgctgcgacaggaggatcacttgagttcgggtcaacccggtatacataggacgtgggggtgggagaagacaaagaagtaaatggtatttaggcccagactgttatacaaaagtgtatttgaagtctacatagtaaatcattggtgttttaagatggaggttttttgtaacatagaggggtaaaaagtagatacttttcttgattagggtgtaaagatcctttgtctcacacaagacaaagcaacagaagaagctactcagttgaaacaaaaagatgcctttgcagcttcggcccttgccgtacgagacgtggagaacccagttagataaagatagtttatgaacaataatttagtttctcacctcatccaatttattgctaagagtttttttggtaaaattctgtcttggaaggcctactggggaaaaagtaagggattttaaacctctttagtgttgtggccatttcttaaaaatgagctaaaatgccctttttgaaagaaatatgattcagaagccatcagaggatcttaaatatggcggtgaggatggaacccattgctgcccacgtgctaggcaagctagcagacacgtgccagcagaccagaaagtgtagcgctgatgatcacagacgaaggacttacgtggtgctgccatccaagcccaatttctcaaactaactgaacatgcttctgttgccatgggtataatataacataggctgggtggttttttgttttgttttgttttttgcctaattttacatggtttatcctgtgaccttcacagcatcatcctacttcctttgcattaggccttgagtgtaaccagcccattgctctacccagtcggagaactgatggttttagtttggggttttttatgggttttgccctagtggttacaaaacaggttttttcttctccttagcactacatgctaagaacacatttgttaccatcccgcccgctctgggatttgtatggaagccagggtgttgagcatgccacttgagcactaagccatgaccttagcctcccacctgcttttgtacaaaagcgtagtttttactgatttgagatgcaccacagtgcacttgggtttgggaacacatttgtaggagtggttttgttgcaccaagtgatcatcaggcctgatttggatggcgcctggcttgaattttatgggatagttctagaggccctgcagcagcccacaccatcctgcccactgcttcaccgataagtccagaattcctcagaagtgatctcttgaaagtgttaaggtttgtggaaaatgtgaattgttttttttttttcccctacagaca

SEQ ID NO: 11 - DNA, 4500 bp, Cricetulus griseus
  source 1..4500: mol_type = genomic DNA
aacacacatcagcatattattggtgaaatcagactgcttgaaatccctaacattcgttaatgaatcattttacaatttccttgttgcttctttgttgaatttaatcccaaagatcttgcttcttcatctatggaaacttaacaccttggactcaataagccttcagtgttacccaaggcctcggaaaccttggtcaggaactgcctggagcaaaatgctaggggttaagagagaaatgcaacttcctgtagctgactagatgatagaataaccaaagcaaaaaaacatatttcaatctctctatgaaagacgatatggaaaatatagaaacaagagacattggcttccagacttacagcccagaagaaacagaaaatacaaccggaagagaggtgctgacttcagccctcccatgaagaaatatgtgcattccagagacttgcagattcttgtagtgtttgagacaggatcgtctcccttggtagcccaagcttgcctcaatatagtagccagttgctttctttctttttttattagtattatatttgggggttggagatggaggtcagaggacagttgacagttctccctttcagcgctgggtcctaggactcgaactcagggtatcaggcatgatggcaggtgcctttgcccagagtcatctcactggctctaagacagctggtttttaatggctatcagtacctttctttctttgagatatggtctcatcattttcttgcctggcttggagctcattatgtagacaaggctagccttgctctcaagagatctgcctgcttccgtctacccagccagagccgtgattaaaccccagatttactttcttgatggaaaaggttaaatgacttcacccgccccttccggtcatttgcctcatcgctgtggaatattactagacttctggcctacataaaaccctaaactcaccgtgctttggtggctcacacctttaatcccagcacttgggaggcagaggcaggcgatctcagtgagttcgaggccagccgggtctacagtacgagttccaggacagcctctaaaacaatacaaagaaacaccaaaacaaaaccctaaactctaaacacaaatacaggcctcaaaaatgcaggtaggtttgatgtagttcactaccagagggaaaagatatattaaatctttcaagaaaggcaccttaacggggaaaagtagtaaattcacgctgcggtggagctgggggagaaaggagggttctaaagggtagggtggagcagctaagtaaagggtgcagcctttacttagcacaagtgggaccctgggttcgatgccctgcacacaacaaccaaatgattaggtaatgttacggggaagttcactttcctttggctacctctgcgtgaggctctccgcagcaaggacaaaaggacagggtcaccttggcgggtggcacccgacagccaggaccaggatccgcgggggtgggggggggtgggggtggggggcacgcagcgcgcaggcgcggtgtcccacacccccctccccgcgccgcgttccacgcgagtgaggctcccacgctgcggcttaacgtttccacgccgctggggtctcccacacctcggggcggggccgggccgcgaaggtcaccaccaaggtcgagagccggacgtgctcgccgcctccaagccgagtgcgtgtgggactcggagtacgtgcggcgggccggagcccgcatgtcggctgcgtagcgacgccccgccctcacccagactccgcagaccctcagctcagcccccggctagcaacgggaggctcgcccagtaggccgaaaatgccacaggcccagccaaccaagtctacccccgcccccgggccatcgtcctcagactgtccgagccaggaggacacctcagtcacgctcttcttctggagtgacagcgccgggggccaatgcccggacggagaggacagagggcgggcccgaaacgccaagaatgggcgggccctcccgagctgctcacaaagtcggagtgggaggcgcttagaccagctcgggaaccggctcgtgcgcacgtccctgctaaacgctctccagggtgtgtataggaacctctgttcttttcctgctcgcccaccggagtgccaggtagggatcgggggcccctggggaacggttcgctcacgagctccgcgtggggggccccggtgggtgtgtgtgcgcccctccagcctgggcgcgtgcccggggactcgggaagcgttcggggcagcctcgtggagggacgtgggctcttggagggggctggggaggtgcagatccacctgttagcatccagacacaggcttgcagggcaactgggctcccaagcctacaaccgcaagtgcagaacagggtggatcgccgcccgggggggttagctaactggaggaaggctttttttttttttttttttttgagggggagaatgatttgacctaatgctcaggaaaaaccttcacaaaatggaagggcctgaaagaaggatgcccaagaggcggtccctcgtcatcgtccgcctccccccccccccccccgggctgctcgcagatcctgctagggctgtggctcatggaccgcaatctagcgtcactgggcgggagtggtccagcccatctctgccacggaatatactccggtgcttattctaggggaaattgcagcagaacccctggatagctggggagggcttaggcgacctcgccccagttaggcaagagttgcgggcttcctgagtggctgctagcaggccgagaaccgacttaggatgtgtttcaggaaatttcctgtcgcccctggcgtaagcagcgtggtccttttgctttcgtgggaggccagagccggcctgggcggatactttgacctctaggtccactattctgccccggctccggccttcagtccacttaaaagacctagagggtgagatttttatcctgggcaaagacagtgcagcccaacttagggatccgagtcagatgcatgctggaaggggagaaccaactcctacacgttagcctgacttcctagtgcgcgctggcacgtgggcgctcccccggcccaaatagatgaaaagaaaactaaagggccattgtgccagacaaggtgatgcgcacatataaacccggcacagggggcgctgcgacaggaggatcacttgagttcgggtcaacccggtatacataggacgtgggggtgggagaagacaaagaagtaaatggtatttaggcccagactgttatacaaaagtgtatttgaagtctacatagtaaatcattggtgttttaagatggaggttttttgtaacatagaggggtaaaaagtagatacttttcttgattagggtgtaaagatcctttgtctcacacaagacaaagcaacagaagaagctactcagttgaaacaaaaagatgcctttgcagcttcggcccttgccgtacgagacgtggagaacccagttagataaagatagtttatgaacaataatttagtttctcacctcatccaatttattgctaagagtttttttggtaaaattctgtcttggaaggcctactggggaaaaagtaagggattttaaacctctttagtgttgtggccatttcttaaaaatgagctaaaatgccctttttgaaagaaatatgattcagaagccatcagaggatcttaaatatggcggtgaggatggaacccattgctgcccacgtgctaggcaagctagcagacacgtgccagcagaccagaaagtgtagcgctgatgatcacagacgaaggacttacgtggtgctgccatccaagcccaatttctcaaactaactgaacatgcttctgttgccatgggtataatataacataggctgggtggttttttgttttgttttgttttttgcctaattttacatggtttatcctgtgaccttcacagcatcatcctacttcctttgcattaggccttgagtgtaaccagcccattgctctacccagtcggagaactgatggttttagtttggggttttttatgggttttgccctagtggttacaaaacaggttttttcttctccttagcactacatgctaagaacacatttgttaccatcccgcccgctctgggatttgtatggaagccagggtgttgagcatgccacttgagcactaagccatgaccttagcctcccacctgcttttgtacaaaagcgtagtttttactgatttgagatgcaccacagtgcacttgggtttgggaacacatttgtaggagtggttttgttgcaccaagtgatcatcaggcctgatttggatggcgcctggcttgaattttatgggatagttctagaggccctgcagcagcccacaccatcctgcccactgcttcaccgataagtccagaattcctcagaagtgatctcttgaaagtgttaaggtttgtggaaaatgtgaattgttttttttttttcccctacagaca

SEQ ID NO: 12 - DNA, 3500 bp, Cricetulus griseus
  source 1..3500: mol_type = genomic DNA
caggcgatctcagtgagttcgaggccagccgggtctacagtacgagttccaggacagcctctaaaacaatacaaagaaacaccaaaacaaaaccctaaactctaaacacaaatacaggcctcaaaaatgcaggtaggtttgatgtagttcactaccagagggaaaagatatattaaatctttcaagaaaggcaccttaacggggaaaagtagtaaattcacgctgcggtggagctgggggagaaaggagggttctaaagggtagggtggagcagctaagtaaagggtgcagcctttacttagcacaagtgggaccctgggttcgatgccctgcacacaacaaccaaatgattaggtaatgttacggggaagttcactttcctttggctacctctgcgtgaggctctccgcagcaaggacaaaaggacagggtcaccttggcgggtggcacccgacagccaggaccaggatccgcgggggtgggggggggtgggggtggggggcacgcagcgcgcaggcgcggtgtcccacacccccctccccgcgccgcgttccacgcgagtgaggctcccacgctgcggcttaacgtttccacgccgctggggtctcccacacctcggggcggggccgggccgcgaaggtcaccaccaaggtcgagagccggacgtgctcgccgcctccaagccgagtgcgtgtgggactcggagtacgtgcggcgggccggagcccgcatgtcggctgcgtagcgacgccccgccctcacccagactccgcagaccctcagctcagcccccggctagcaacgggaggctcgcccagtaggccgaaaatgccacaggcccagccaaccaagtctacccccgcccccgggccatcgtcctcagactgtccgagccaggaggacacctcagtcacgctcttcttctggagtgacagcgccgggggccaatgcccggacggagaggacagagggcgggcccgaaacgccaagaatgggcgggccctcccgagctgctcacaaagtcggagtgggaggcgcttagaccagctcgggaaccggctcgtgcgcacgtccctgctaaacgctctccagggtgtgtataggaacctctgttcttttcctgctcgcccaccggagtgccaggtagggatcgggggcccctggggaacggttcgctcacgagctccgcgtggggggccccggtgggtgtgtgtgcgcccctccagcctgggcgcgtgcccggggactcgggaagcgttcggggcagcctcgtggagggacgtgggctcttggagggggctggggaggtgcagatccacctgttagcatccagacacaggcttgcagggcaactgggctcccaagcctacaaccgcaagtgcagaacagggtggatcgccgcccgggggggttagctaactggaggaaggctttttttttttttttttttttgagggggagaatgatttgacctaatgctcaggaaaaaccttcacaaaatggaagggcctgaaagaaggatgcccaagaggcggtccctcgtcatcgtccgcctccccccccccccccccgggctgctcgcagatcctgctagggctgtggctcatggaccgcaatctagcgtcactgggcgggagtggtccagcccatctctgccacggaatatactccggtgcttattctaggggaaattgcagcagaacccctggatagctggggagggcttaggcgacctcgccccagttaggcaagagttgcgggcttcctgagtggctgctagcaggccgagaaccgacttaggatgtgtttcaggaaatttcctgtcgcccctggcgtaagcagcgtggtccttttgctttcgtgggaggccagagccggcctgggcggatactttgacctctaggtccactattctgccccggctccggccttcagtccacttaaaagacctagagggtgagatttttatcctgggcaaagacagtgcagcccaacttagggatccgagtcagatgcatgctggaaggggagaaccaactcctacacgttagcctgacttcctagtgcgcgctggcacgtgggcgctcccccggcccaaatagatgaaaagaaaactaaagggccattgtgccagacaaggtgatgcgcacatataaacccggcacagggggcgctgcgacaggaggatcacttgagttcgggtcaacccggtatacataggacgtgggggtgggagaagacaaagaagtaaatggtatttaggcccagactgttatacaaaagtgtatttgaagtctacatagtaaatcattggtgttttaagatggaggttttttgtaacatagaggggtaaaaagtagatacttttcttgattagggtgtaaagatcctttgtctcacacaagacaaagcaacagaagaagctactcagttgaaacaaaaagatgcctttgcagcttcggcccttgccgtacgagacgtggagaacccagttagataaagatagtttatgaacaataatttagtttctcacctcatccaatttattgctaagagtttttttggtaaaattctgtcttggaaggcctactggggaaaaagtaagggattttaaacctctttagtgttgtggccatttcttaaaaatgagctaaaatgccctttttgaaagaaatatgattcagaagccatcagaggatcttaaatatggcggtgaggatggaacccattgctgcccacgtgctaggcaagctagcagacacgtgccagcagaccagaaagtgtagcgctgatgatcacagacgaaggacttacgtggtgctgccatccaagcccaatttctcaaactaactgaacatgcttctgttgccatgggtataatataacataggctgggtggttttttgttttgttttgttttttgcctaattttacatggtttatcctgtgaccttcacagcatcatcctacttcctttgcattaggccttgagtgtaaccagcccattgctctacccagtcggagaactgatggttttagtttggggttttttatgggttttgccctagtggttacaaaacaggttttttcttctccttagcactacatgctaagaacacatttgttaccatcccgcccgctctgggatttgtatggaagccagggtgttgagcatgccacttgagcactaagccatgaccttagcctcccacctgcttttgtacaaaagcgtagtttttactgatttgagatgcaccacagtgcacttgggtttgggaacacatttgtaggagtggttttgttgcaccaagtgatcatcaggcctgatttggatggcgcctggcttgaattttatgggatagttctagaggccctgcagcagcccacaccatcctgcccactgcttcaccgataagtccagaattcctcagaagtgatctcttgaaagtgttaaggtttgtggaaaatgtgaattgttttttttttttcccctacagaca

SEQ ID NO: 13 - DNA, 2707 bp, Cricetulus griseus
  source 1..2707: mol_type = genomic DNA
ggctagcaacgggaggctcgcccagtaggccgaaaatgccacaggcccagccaaccaagtctacccccgcccccgggccatcgtcctcagactgtccgagccaggaggacacctcagtcacgctcttcttctggagtgacagcgccgggggccaatgcccggacggagaggacagagggcgggcccgaaacgccaagaatgggcgggccctcccgagctgctcacaaagtcggagtgggaggcgcttagaccagctcgggaaccggctcgtgcgcacgtccctgctaaacgctctccagggtgtgtataggaacctctgttcttttcctgctcgcccaccggagtgccaggtagggatcgggggcccctggggaacggttcgctcacgagctccgcgtggggggccccggtgggtgtgtgtgcgcccctccagcctgggcgcgtgcccggggactcgggaagcgttcggggcagcctcgtggagggacgtgggctcttggagggggctggggaggtgcagatccacctgttagcatccagacacaggcttgcagggcaactgggctcccaagcctacaaccgcaagtgcagaacagggtggatcgccgcccgggggggttagctaactggaggaaggctttttttttttttttttttttgagggggagaatgatttgacctaatgctcaggaaaaaccttcacaaaatggaagggcctgaaagaaggatgcccaagaggcggtccctcgtcatcgtccgcctccccccccccccccccgggctgctcgcagatcctgctagggctgtggctcatggaccgcaatctagcgtcactgggcgggagtggtccagcccatctctgccacggaatatactccggtgcttattctaggggaaattgcagcagaacccctggatagctggggagggcttaggcgacctcgccccagttaggcaagagttgcgggcttcctgagtggctgctagcaggccgagaaccgacttaggatgtgtttcaggaaatttcctgtcgcccctggcgtaagcagcgtggtccttttgctttcgtgggaggccagagccggcctgggcggatactttgacctctaggtccactattctgccccggctccggccttcagtccacttaaaagacctagagggtgagatttttatcctgggcaaagacagtgcagcccaacttagggatccgagtcagatgcatgctggaaggggagaaccaactcctacacgttagcctgacttcctagtgcgcgctggcacgtgggcgctcccccggcccaaatagatgaaaagaaaactaaagggccattgtgccagacaaggtgatgcgcacatataaacccggcacagggggcgctgcgacaggaggatcacttgagttcgggtcaacccggtatacataggacgtgggggtgggagaagacaaagaagtaaatggtatttaggcccagactgttatacaaaagtgtatttgaagtctacatagtaaatcattggtgttttaagatggaggttttttgtaacatagaggggtaaaaagtagatacttttcttgattagggtgtaaagatcctttgtctcacacaagacaaagcaacagaagaagctactcagttgaaacaaaaagatgcctttgcagcttcggcccttgccgtacgagacgtggagaacccagttagataaagatagtttatgaacaataatttagtttctcacctcatccaatttattgctaagagtttttttggtaaaattctgtcttggaaggcctactggggaaaaagtaagggattttaaacctctttagtgttgtggccatttcttaaaaatgagctaaaatgccctttttgaaagaaatatgattcagaagccatcagaggatcttaaatatggcggtgaggatggaacccattgctgcccacgtgctaggcaagctagcagacacgtgccagcagaccagaaagtgtagcgctgatgatcacagacgaaggacttacgtggtgctgccatccaagcccaatttctcaaactaactgaacatgcttctgttgccatgggtataatataacataggctgggtggttttttgttttgttttgttttttgcctaattttacatggtttatcctgtgaccttcacagcatcatcctacttcctttgcattaggccttgagtgtaaccagcccattgctctacccagtcggagaactgatggttttagtttggggttttttatgggttttgccctagtggttacaaaacaggttttttcttctccttagcactacatgctaagaacacatttgttaccatcccgcccgctctgggatttgtatggaagccagggtgttgagcatgccacttgagcactaagccatgaccttagcctcccacctgcttttgtacaaaagcgtagtttttactgatttgagatgcaccacagtgcacttgggtttgggaacacatttgtaggagtggttttgttgcaccaagtgatcatcaggcctgatttggatggcgcctggcttgaattttatgggatagttctagaggccctgcagcagcccacaccatcctgcccactgcttcaccgataagtccagaattcctcagaagtgatctcttgaaagtgttaaggtttgtggaaaatgtgaattgttttttttttttcccctacagaca

SEQ ID NO: 14 - DNA, 2607 bp, Cricetulus griseus
  source 1..2607: mol_type = genomic DNA
ccaggaggacacctcagtcacgctcttcttctggagtgacagcgccgggggccaatgcccggacggagaggacagagggcgggcccgaaacgccaagaatgggcgggccctcccgagctgctcacaaagtcggagtgggaggcgcttagaccagctcgggaaccggctcgtgcgcacgtccctgctaaacgctctccagggtgtgtataggaacctctgttcttttcctgctcgcccaccggagtgccaggtagggatcgggggcccctggggaacggttcgctcacgagctccgcgtggggggccccggtgggtgtgtgtgcgcccctccagcctgggcgcgtgcccggggactcgggaagcgttcggggcagcctcgtggagggacgtgggctcttggagggggctggggaggtgcagatccacctgttagcatccagacacaggcttgcagggcaactgggctcccaagcctacaaccgcaagtgcagaacagggtggatcgccgcccgggggggttagctaactggaggaaggctttttttttttttttttttttgagggggagaatgatttgacctaatgctcaggaaaaaccttcacaaaatggaagggcctgaaagaaggatgcccaagaggcggtccctcgtcatcgtccgcctccccccccccccccccgggctgctcgcagatcctgctagggctgtggctcatggaccgcaatctagcgtcactgggcgggagtggtccagcccatctctgccacggaatatactccggtgcttattctaggggaaattgcagcagaacccctggatagctggggagggcttaggcgacctcgccccagttaggcaagagttgcgggcttcctgagtggctgctagcaggccgagaaccgacttaggatgtgtttcaggaaatttcctgtcgcccctggcgtaagcagcgtggtccttttgctttcgtgggaggccagagccggcctgggcggatactttgacctctaggtccactattctgccccggctccggccttcagtccacttaaaagacctagagggtgagatttttatcctgggcaaagacagtgcagcccaacttagggatccgagtcagatgcatgctggaaggggagaaccaactcctacacgttagcctgacttcctagtgcgcgctggcacgtgggcgctcccccggcccaaatagatgaaaagaaaactaaagggccattgtgccagacaaggtgatgcgcacatataaacccggcacagggggcgctgcgacaggaggatcacttgagttcgggtcaacccggtatacataggacgtgggggtgggagaagacaaagaagtaaatggtatttaggcccagactgttatacaaaagtgtatttgaagtctacatagtaaatcattggtgttttaagatggaggttttttgtaacatagaggggtaaaaagtagatacttttcttgattagggtgtaaagatcctttgtctcacacaagacaaagcaacagaagaagctactcagttgaaacaaaaagatgcctttgcagcttcggcccttgccgtacgagacgtggagaacccagttagataaagatagtttatgaacaataatttagtttctcacctcatccaatttattgctaagagtttttttggtaaaattctgtcttggaaggcctactggggaaaaagtaagggattttaaacctctttagtgttgtggccatttcttaaaaatgagctaaaatgccctttttgaaagaaatatgattcagaagccatcagaggatcttaaatatggcggtgaggatggaacccattgctgcccacgtgctaggcaagctagcagacacgtgccagcagaccagaaagtgtagcgctgatgatcacagacgaaggacttacgtggtgctgccatccaagcccaatttctcaaactaactgaacatgcttctgttgccatgggtataatataacataggctgggtggttttttgttttgttttgttttttgcctaattttacatggtttatcctgtgaccttcacagcatcatcctacttcctttgcattaggccttgagtgtaaccagcccattgctctacccagtcggagaactgatggttttagtttggggttttttatgggttttgccctagtggttacaaaacaggttttttcttctccttagcactacatgctaagaacacatttgttaccatcccgcccgctctgggatttgtatggaagccagggtgttgagcatgccacttgagcactaagccatgaccttagcctcccacctgcttttgtacaaaagcgtagtttttactgatttgagatgcaccacagtgcacttgggtttgggaacacatttgtaggagtggttttgttgcaccaagtgatcatcaggcctgatttggatggcgcctggcttgaattttatgggatagttctagaggccctgcagcagcccacaccatcctgcccactgcttcaccgataagtccagaattcctcagaagtgatctcttgaaagtgttaaggtttgtggaaaatgtgaattgttttttttttttcccctacagaca

SEQ ID NO: 15 - DNA, 2507 bp, Cricetulus griseus
  source 1..2507: mol_type = genomic DNA
gggcgggccctcccgagctgctcacaaagtcggagtgggaggcgcttagaccagctcgggaaccggctcgtgcgcacgtccctgctaaacgctctccagggtgtgtataggaacctctgttcttttcctgctcgcccaccggagtgccaggtagggatcgggggcccctggggaacggttcgctcacgagctccgcgtggggggccccggtgggtgtgtgtgcgcccctccagcctgggcgcgtgcccggggactcgggaagcgttcggggcagcctcgtggagggacgtgggctcttggagggggctggggaggtgcagatccacctgttagcatccagacacaggcttgcagggcaactgggctcccaagcctacaaccgcaagtgcagaacagggtggatcgccgcccgggggggttagctaactggaggaaggctttttttttttttttttttttgagggggagaatgatttgacctaatgctcaggaaaaaccttcacaaaatggaagggcctgaaagaaggatgcccaagaggcggtccctcgtcatcgtccgcctccccccccccccccccgggctgctcgcagatcctgctagggctgtggctcatggaccgcaatctagcgtcactgggcgggagtggtccagcccatctctgccacggaatatactccggtgcttattctaggggaaattgcagcagaacccctggatagctggggagggcttaggcgacctcgccccagttaggcaagagttgcgggcttcctgagtggctgctagcaggccgagaaccgacttaggatgtgtttcaggaaatttcctgtcgcccctggcgtaagcagcgtggtccttttgctttcgtgggaggccagagccggcctgggcggatactttgacctctaggtccactattctgccccggctccggccttcagtccacttaaaagacctagagggtgagatttttatcctgggcaaagacagtgcagcccaacttagggatccgagtcagatgcatgctggaaggggagaaccaactcctacacgttagcctgacttcctagtgcgcgctggcacgtgggcgctcccccggcccaaatagatgaaaagaaaactaaagggccattgtgccagacaaggtgatgcgcacatataaacccggcacagggggcgctgcgacaggaggatcacttgagttcgggtcaacccggtatacataggacgtgggggtgggagaagacaaagaagtaaatggtatttaggcccagactgttatacaaaagtgtatttgaagtctacatagtaaatcattggtgttttaagatggaggttttttgtaacatagaggggtaaaaagtagatacttttcttgattagggtgtaaagatcctttgtctcacacaagacaaagcaacagaagaagctactcagttgaaacaaaaagatgcctttgcagcttcggcccttgccgtacgagacgtggagaacccagttagataaagatagtttatgaacaataatttagtttctcacctcatccaatttattgctaagagtttttttggtaaaattctgtcttggaaggcctactggggaaaaagtaagggattttaaacctctttagtgttgtggccatttcttaaaaatgagctaaaatgccctttttgaaagaaatatgattcagaagccatcagaggatcttaaatatggcggtgaggatggaacccattgctgcccacgtgctaggcaagctagcagacacgtgccagcagaccagaaagtgtagcgctgatgatcacagacgaaggacttacgtggtgctgccatccaagcccaatttctcaaactaactgaacatgcttctgttgccatgggtataatataacataggctgggtggttttttgttttgttttgttttttgcctaattttacatggtttatcctgtgaccttcacagcatcatcctacttcctttgcattaggccttgagtgtaaccagcccattgctctacccagtcggagaactgatggttttagtttggggttttttatgggttttgccctagtggttacaaaacaggttttttcttctccttagcactacatgctaagaacacatttgttaccatcccgcccgctctgggatttgtatggaagccagggtgttgagcatgccacttgagcactaagccatgaccttagcctcccacctgcttttgtacaaaagcgtagtttttactgatttgagatgcaccacagtgcacttgggtttgggaacacatttgtaggagtggttttgttgcaccaagtgatcatcaggcctgatttggatggcgcctggcttgaattttatgggatagttctagaggccctgcagcagcccacaccatcctgcccactgcttcaccgataagtccagaattcctcagaagtgatctcttgaaagtgttaaggtttgtggaaaatgtgaattgttttttttttttcccctacagaca

SEQ ID NO: 16 - DNA, 4000 bp, Mus musculus
  source 1..4000: mol_type = genomic DNA
taactcccagactcacaacccaagagaaacgtgggagaaaatacaacagaaagtgatgtgttcccttcagttctatagtgaagtgtgtgcacggcaggagttgaaagccgatttctgtagtgtttgagatgagatcgggtccctaggcagctcaagtttgtctcgatttgatggctactttttttcttttgattagtattacacattgtggttggggatggaggtcagaggacagcttgatcaggtgtgactgactgcaggtgcctttgcccctgagccatctcgtgggttccaagatagggttttgtttgtctgtcttattttaaaatattgtttggttttgggtttgtttgtttggttttttttggacagggtttctccttgtaacttatctgttcaggaactagctctgtagattaaaggctcacattagcactgactggctagctatcatcacttttattttttctcttttcttcatttctttctttttctcttttcttttcttttctttctttctttctttctttctttctttctttctctttcttttttttttttttttgacaaggtctcatcactatgccccatctgaattagaattcactatgtagaccaggcaggccttgaactcagaaatccgcctgcctctgcctacccacagctgtggttaaacaccagctttattttcttcatcagaagggtgaaatggctccaccctgcgcttccggacgtttgtcacatcattgtggaatattactagtctagacttttgagaaatgcgtcgggacgacttgagtatgagtctcaagaactggtaggtcaagaacatcgaggccacaagcaggggaaagaagtattagatctttaaacaaaggaacattaacatggatgaagaataaatccacactgagctagtacaccagagaagtaaggaaagttctaaagtagggtggagtggctgggtgggtgtagcacaaaggtactgccttattagcgtgagctggacagtaggattcggtaccctccacacagtaacaaatgattaggtaatattaagggaaaggtcactttcccttggctacctcggcctgagactcactacagcaaggacaaaaggacggggtcaccttggcagatggcaccagagagccaggaccagcggcgagggcgctcagtgcgcaggcgcagtatccatgcatttccccctcatcccccccacccccacccaattccacgcgggagtgaggccctctggccgcgcatcaacgtttccacaccgccgggggctccagaacctcccggtggggggttggccggctggagggccgagccgcgaaggtcatcagcaaggtcgtgggccggacgtgtggcgccgcagccacgccgagtgcgtgtgagactcggagtacgtgcggcgggctcaagccctcatgcccgccgcgcagcccagccccgccccgccccgcatccgggctccgtagaccctcggccgggccccaggttcccagccggaggctcgccaggcattccagctatgccccaagcaggctaggcccagaaaggcaggacaacccccgcccccgtgccctcgcccctagtctgggcaggccgagcggccgcctcggtcacgctcttctattggagtgatggcacgctgagccaatggggaggcggcgcggagggagggcgggcccgaaaggggagaactgggcggggcttaacgagcaggaaaggaagacagagtgggaggcgcttagtgctgctccggtacagggtcgcgctcgcgtctgtccttaaggctctcctcggtgtccacggcaccctctttccttgctttgcagcgatcctactgccaggtatggtccttgtctccaccggggtcagctctcctactagcttcgcttggggacccggtgggcacgtgcacccactagcctgggcgggagccgctatccggggagcactcgggtcagcctcgtggaaggacgcaggctcttggagggtggaggtgtgagccccaccagtgatcaccgagtttcagggttgcaatgtaaccgggttcccaagcagacaacagcaaatgcagaccacggatgatcgcggccgtggagaatagaaaagtactttctgtgtagttaagtggaaggtttcagagggagggagagcaacttaaacccccgatgctcattaaatcctttctcagaatggaagggccagaaataaggatgcccaagaggcagagcgccacaccctagtagatcctgctggggctgtagctcctggaccgcaatcgagcgtcactgggcgggagtggtccagcccatctctgctgtggaatattcctgacctgtgagtgtcggttaggtactaagagtagaggaaattgcagcagtcccgttggataattgggaagccctcaggagacctcgacgcaattaggcaagagctacaggtttcctgggtggctactagccggccgtgaactgacttaagatgcatttaagaaaacttcctgttcgttctggcctaggcagtgtggttccttggctgactcgctttcgggatagaccacagctagtctgctgattagcctgaccgataggtccacttttctgcccttggtctggcgttcaatccagataaagacagagtgggtgagattttcttcctttggttaaatacgtttgctgcctagcctaaagatccaagctagataaaaagggtggagggagggatcaactcctacaagttgtaaggtctttgcagagcaaagtgtggcacgtgggtgctcctccgcccccataaaggaaccagccatggagatgcacacatgaaagtgtagcgctagggatgctgaggctggaggatcactgagttctggtcagtctggcattcatagaatcgggcgagtaagagagaagacaaaagagtatggttgaggaatagtaaggttttgtaacatggtaggtaaaaagtagatactttattcttggtgagtgtacaaagatcctttgtcttagagaagacaaaaccacagaagtaacttctgtggaaaaaaaagctgcctttgcttcagtgcttgccacaaaagatgtgaggaacctagttagataataatagcctctgaatgctgtattgtcttcatgtctcatccagtttagctacagaatctatttggtttctttcttggaaagcctgctggggaagaagtaagaaagggacttgcagtttgttgccaaatatcctcttcctctcaggatgtttttctaattaaacatctactttgaataccttttaaaagcgagacaaggtgcccttttgaaatgtactaaccagaagtcctagctcttgcctaaatatggcggagattgaacccaggacctcccacgtgctagccagcatggccaccaggccaagaatggcaggatcattgaccacaggccaaggagtttggggttctggcctcctgcctcacactttcttactggttatcaaatctgtgtcagctgaatattctgctcttgtcatgggtgcaatttgatgaattagggtttctctttttcccacaattaaactgctttgaaatgtcacatttccctctggtctccaggtcagtttaacctctgaccttccttcactgttgcttcccacttccttctctgtggagccagaacactgttctatgcagtcagaggatttaatttgcccacagtacaggtagcttctgagggctttctgtaggagtggtttatttcattgtgccatgttgacctcaagcttggcgggaagtccaagccaccgacctgctgtgtaaggagtagtcctcgctccccaaaccctcactgatgagtgactttcctgtatgttacctaacgcatagcccatttggtacctgtcaagtccaggacccctcagaggtgatggccttggaatgaattaacctctgtgtcactgtttattggtgatatgaatgtttttcctcctacagaaattcgcc

SEQ ID NO: 17 - DNA, 3500 bp, Mus musculus
  source 1..3500: mol_type = genomic DNA
cttttcttttctttctttctttctttctttctttctttctttctctttcttttttttttttttttgacaaggtctcatcactatgccccatctgaattagaattcactatgtagaccaggcaggccttgaactcagaaatccgcctgcctctgcctacccacagctgtggttaaacaccagctttattttcttcatcagaagggtgaaatggctccaccctgcgcttccggacgtttgtcacatcattgtggaatattactagtctagacttttgagaaatgcgtcgggacgacttgagtatgagtctcaagaactggtaggtcaagaacatcgaggccacaagcaggggaaagaagtattagatctttaaacaaaggaacattaacatggatgaagaataaatccacactgagctagtacaccagagaagtaaggaaagttctaaagtagggtggagtggctgggtgggtgtagcacaaaggtactgccttattagcgtgagctggacagtaggattcggtaccctccacacagtaacaaatgattaggtaatattaagggaaaggtcactttcccttggctacctcggcctgagactcactacagcaaggacaaaaggacggggtcaccttggcagatggcaccagagagccaggaccagcggcgagggcgctcagtgcgcaggcgcagtatccatgcatttccccctcatcccccccacccccacccaattccacgcgggagtgaggccctctggccgcgcatcaacgtttccacaccgccgggggctccagaacctcccggtggggggttggccggctggagggccgagccgcgaaggtcatcagcaaggtcgtgggccggacgtgtggcgccgcagccacgccgagtgcgtgtgagactcggagtacgtgcggcgggctcaagccctcatgcccgccgcgcagcccagccccgccccgccccgcatccgggctccgtagaccctcggccgggccccaggttcccagccggaggctcgccaggcattccagctatgccccaagcaggctaggcccagaaaggcaggacaacccccgcccccgtgccctcgcccctagtctgggcaggccgagcggccgcctcggtcacgctcttctattggagtgatggcacgctgagccaatggggaggcggcgcggagggagggcgggcccgaaaggggagaactgggcggggcttaacgagcaggaaaggaagacagagtgggaggcgcttagtgctgctccggtacagggtcgcgctcgcgtctgtccttaaggctctcctcggtgtccacggcaccctctttccttgctttgcagcgatcctactgccaggtatggtccttgtctccaccggggtcagctctcctactagcttcgcttggggacccggtgggcacgtgcacccactagcctgggcgggagccgctatccggggagcactcgggtcagcctcgtggaaggacgcaggctcttggagggtggaggtgtgagccccaccagtgatcaccgagtttcagggttgcaatgtaaccgggttcccaagcagacaacagcaaatgcagaccacggatgatcgcggccgtggagaatagaaaagtactttctgtgtagttaagtggaaggtttcagagggagggagagcaacttaaacccccgatgctcattaaatcctttctcagaatggaagggccagaaataaggatgcccaagaggcagagcgccacaccctagtagatcctgctggggctgtagctcctggaccgcaatcgagcgtcactgggcgggagtggtccagcccatctctgctgtggaatattcctgacctgtgagtgtcggttaggtactaagagtagaggaaattgcagcagtcccgttggataattgggaagccctcaggagacctcgacgcaattaggcaagagctacaggtttcctgggtggctactagccggccgtgaactgacttaagatgcatttaagaaaacttcctgttcgttctggcctaggcagtgtggttccttggctgactcgctttcgggatagaccacagctagtctgctgattagcctgaccgataggtccacttttctgcccttggtctggcgttcaatccagataaagacagagtgggtgagattttcttcctttggttaaatacgtttgctgcctagcctaaagatccaagctagataaaaagggtggagggagggatcaactcctacaagttgtaaggtctttgcagagcaaagtgtggcacgtgggtgctcctccgcccccataaaggaaccagccatggagatgcacacatgaaagtgtagcgctagggatgctgaggctggaggatcactgagttctggtcagtctggcattcatagaatcgggcgagtaagagagaagacaaaagagtatggttgaggaatagtaaggttttgtaacatggtaggtaaaaagtagatactttattcttggtgagtgtacaaagatcctttgtcttagagaagacaaaaccacagaagtaacttctgtggaaaaaaaagctgcctttgcttcagtgcttgccacaaaagatgtgaggaacctagttagataataatagcctctgaatgctgtattgtcttcatgtctcatccagtttagctacagaatctatttggtttctttcttggaaagcctgctggggaagaagtaagaaagggacttgcagtttgttgccaaatatcctcttcctctcaggatgtttttctaattaaacatctactttgaataccttttaaaagcgagacaaggtgcccttttgaaatgtactaaccagaagtcctagctcttgcctaaatatggcggagattgaacccaggacctcccacgtgctagccagcatggccaccaggccaagaatggcaggatcattgaccacaggccaaggagtttggggttctggcctcctgcctcacactttcttactggttatcaaatctgtgtcagctgaatattctgctcttgtcatgggtgcaatttgatgaattagggtttctctttttcccacaattaaactgctttgaaatgtcacatttccctctggtctccaggtcagtttaacctctgaccttccttcactgttgcttcccacttccttctctgtggagccagaacactgttctatgcagtcagaggatttaatttgcccacagtacaggtagcttctgagggctttctgtaggagtggtttatttcattgtgccatgttgacctcaagcttggcgggaagtccaagccaccgacctgctgtgtaaggagtagtcctcgctccccaaaccctcactgatgagtgactttcctgtatgttacctaacgcatagcccatttggtacctgtcaagtccaggacccctcagaggtgatggccttggaatgaattaacctctgtgtcactgtttattggtgatatgaatgtttttcctcctacagaaattcgcc

SEQ ID NO: 18 - DNA, 100 bp, Cricetulus griseus
  source 1..100: mol_type = genomic DNA
gtgggactcggagtacgtgcggcgggccggagcccgcatgtcggctgcgtagcgacgccccgccctcacccagactccgcagaccctcagctcagccccc